European Patent Specification EP 4 082 558 B1, published August 23, 2023. Title: TOXIN-DERIVED DELIVERY CONSTRUCTS FOR ORAL DELIVERY. Applicant: APPLIED MOLECULAR TRANSPORT INC. The sequence listing filed with the application follows.

SEQUENCE LISTING (221 sequences)

SEQ ID NO: 1 - protein, 634 aa, Vibrio cholera
VEEALNIFDECRSPCSLTPEPGKPIQSKLSIPSDVVLDEGVLYYSMTINDEQNDIKDEDKGESIITIGEFATVRATRHYVNQDAPFGVIHLDITTENGTKTYSYNRKEGEFAINWLVPIGEDSPASIKISVDELDQQRNIIEVPKLYSIDLDNQTLEQWKTQGNVSFSVTRPEHNIAISWPSVSYKAAQKEGSRHKRWAHWHTGLALCWLVPMDAIYNYITQQNCTLGDNWFGGSYETVAGTPKVITVKQGIEQKPVEQRIHFSKGNAMSALAAHRVCGVPLETLARSRKPRDLTDDLSCAYQAQNIVSLFVATRILFSHLDSVFTLNLDEQEPEVAERLSDLRRINENNPGMVTQVLTVARQIYNDYVTHHPGLTPEQTSAGAQAADILSLFCPDADKSCVASNNDQANINIESRSGRSYLPENRAVITPQGVTNWTYQELEATHQALTREGYVFVGYHGTNHVAAQTIVNRIAPVPRGNNTENEEKWGGLYVATHAEVAHGYARIKEGTGEYGLPTRAERDARGVMLRVYIPRASLERFYRTNTPLENAEEHITQVIGHSLPLRNEAFTGPESAGGEDETVIGWDMAIHAVAIPSTIPGNAYEELAIDEEAVAKEQSISTKPPYKERKDELK

SEQ ID NO: 2 - protein, 634 aa, Vibrio cholera
VEDELNIFDECRSPCSLTPEPGKPIQSKLSIPSDVVLDEGVLYYSMTINDEQNDIKDEDKGESIITIGEFATVRATRHYVNQDAPFGVIHLDITTENGTKTYSYNRKEGEFAINWLVPIGEDSPASIKISVDELDQQRNIIEVPKLYSIDLDNQTLEQWKTQGNVSFSVTRPEHNIAISWPSVSYKAAQKEGSRHKRWAHWHTGLALCWLVPMDAIYNYITQQNCTLGDNWFGGSYETVAGTPKVITVKQGIEQKPVEQRIHFSKGNAMSALAAHRVCGVPLETLARSRKPRDLTDDLSCAYQAQNIVSLFVATRILFSHLDSVFTLNLDEQEPEVAERLSDLRRINENNPGMVTQVLTVARQIYNDYVTHHPGLTPEQTSAGAQAADILSLFCPDADKSCVASNNDQANINIESRSGRSYLPENRAVITPQGVTNWTYQELEATHQALTREGYVFVGYHGTNHVAAQTIVNRIAPVPRGNNTENEEKWGGLYVATHAEVAHGYARIKEGTGEYGLPTRAERDARGVMLRVYIPRASLERFYRTNTPLENAEEHITQVIGHSLPLRNEAFTGPESAGGEDETVIGWDMAIHAVAIPSTIPGNAYEELAIDEEAVAKEQSISTKPPYKERKDELK

SEQ ID NO: 3 - protein, 634 aa, Vibrio cholera
VEDELNIFDECRSPCSLTPEPGKPIQSKLSIPSDVVLDEGVLYYSMTINDEQNDIKDEDKGESIITIGEFATVRATRHYVNQDAPFGVIHLDITTENGTKTYSYNRKEGEFAINWLVPIGEDSPASIKISVDELDQQRNIIEVPKLYSIDLDNQTLEQWKTQGNVSFSVTRPEHNIAISWPSVSYKAAQKEGSRHKRWAHWHTGLALCWLVPMDAIYNYITQQNCTLGDNWFGGSYETVAGTPKVITVKQGIEQKPVEQRIHFSKGNAMSALAAHRVCGVPLETLARSRKPRDLTDDLSCAYQAQNIVSLFVATRILFSHLDSVFTLNLDEQEPEVAERLSDLRRINENNPGMVTQVLTVARQIYNDYVTHHPGLTPEQTSAGAQAADILSLFCPDADKSCVASNNDQANINIESRSGRSYLPENRAVITPQGVTNWTYQELEATHQALTREGYVFVGYHGTNHVAAQTIVNRIAPVPRGNNTENEEKWGGLYVATHAEVAHGYARIKEGTGEYGLPTRAERDARGVMLRVYIPRASLERFYRTNTPLENAEEHITQVIGHSLPLRNEAFTGPESAGGEDATVIGWDMAIHAVAIPSTIPGNAYEELAIDEEAVAKEQSISTKPPYKERKDELK

SEQ ID NO: 4 - protein, 265 aa, Vibrio cholera
VEEALNIFDECRSPCSLTPEPGKPIQSKLSIPSDVVLDEGVLYYSMTINDEQNDIKDEDKGESIITIGEFATVRATRHYVNQDAPFGVIHLDITTENGTKTYSYNRKEGEFAINWLVPIGEDSPASIKISVDELDQQRNIIEVPKLYSIDLDNQTLEQWKTQGNVSFSVTRPEHNIAISWPSVSYKAAQKEGSRHKRWAHWHTGLALCWLVPMDAIYNYITQQNCTLGDNWFGGSYETVAGTPKVITVKQGIEQKPVEQRIHFSK

SEQ ID NO: 5 - protein, 266 aa, Artificial Sequence
  source: /note="Description of Artificial Sequence: Synthetic polypeptide"
MVEEALNIFDECRSPCSLTPEPGKPIQSKLSIPSDVVLDEGVLYYSMTINDEQNDIKDEDKGESIITIGEFATVRATRHYVNQDAPFGVIHLDITTENGTKTYSYNRKEGEFAINWLVPIGEDSPASIKISVDELDQQRNIIEVPKLYSIDLDNQTLEQWKTQGNVSFSVTRPEHNIAISWPSVSYKAAQKEGSRHKRWAHWHTGLALCWLVPMDAIYNYITQQNCTLGDNWFGGSYETVAGTPKVITVKQGIEQKPVEQRIHFSK

SEQ ID NO: 6 - protein, 250 aa, Vibrio cholera
VEEALNIFDECRSPCSLTPEPGKPIQSKLSIPSDVVLDEGVLYYSMTINDEQNDIKDEDKGESIITIGEFATVRATRHYVNQDAPFGVIHLDITTENGTKTYSYNRKEGEFAINWLVPIGEDSPASIKISVDELDQQRNIIEVPKLYSIDLDNQTLEQWKTQGNVSFSVTRPEHNIAISWPSVSYKAAQKEGSRHKRWAHWHTGLALCWLVPMDAIYNYITQQNCTLGDNWFGGSYETVAGTPKVITVKQ

SEQ ID NO: 7 - protein, 251 aa, Artificial Sequence
  source: /note="Description of Artificial Sequence: Synthetic polypeptide"
MVEEALNIFDECRSPCSLTPEPGKPIQSKLSIPSDVVLDEGVLYYSMTINDEQNDIKDEDKGESIITIGEFATVRATRHYVNQDAPFGVIHLDITTENGTKTYSYNRKEGEFAINWLVPIGEDSPASIKISVDELDQQRNIIEVPKLYSIDLDNQTLEQWKTQGNVSFSVTRPEHNIAISWPSVSYKAAQKEGSRHKRWAHWHTGLALCWLVPMDAIYNYITQQNCTLGDNWFGGSYETVAGTPKVITVKQ

SEQ ID NO: 8 - protein, 244 aa, Vibrio cholera
VEEALNIFDECRSPCSLTPEPGKPIQSKLSIPSDVVLDEGVLYYSMTINDEQNDIKDEDKGESIITIGEFATVRATRHYVNQDAPFGVIHLDITTENGTKTYSYNRKEGEFAINWLVPIGEDSPASIKISVDELDQQRNIIEVPKLYSIDLDNQTLEQWKTQGNVSFSVTRPEHNIAISWPSVSYKAAQKEGSRHKRWAHWHTGLALCWLVPMDAIYNYITQQNCTLGDNWFGGSYETVAGTPK

SEQ ID NO: 9 - protein, 245 aa, Artificial Sequence
  source: /note="Description of Artificial Sequence: Synthetic polypeptide"
MVEEALNIFDECRSPCSLTPEPGKPIQSKLSIPSDVVLDEGVLYYSMTINDEQNDIKDEDKGESIITIGEFATVRATRHYVNQDAPFGVIHLDITTENGTKTYSYNRKEGEFAINWLVPIGEDSPASIKISVDELDQQRNIIEVPKLYSIDLDNQTLEQWKTQGNVSFSVTRPEHNIAISWPSVSYKAAQKEGSRHKRWAHWHTGLALCWLVPMDAIYNYITQQNCTLGDNWFGGSYETVAGTPK

SEQ ID NO: 10 - protein, 205 aa, Vibrio cholera
VEEALNIFDECRSPCSLTPEPGKPIQSKLSIPSDVVLDEGVLYYSMTINDEQNDIKDEDKGESIITIGEFATVRATRHYVNQDAPFGVIHLDITTENGTKTYSYNRKEGEFAINWLVPIGEDSPASIKISVDELDQQRNIIEVPKLYSIDLDNQTLEQWKTQGNVSFSVTRPEHNIAISWPSVSYKAAQKEGSRHKRWAHWHTGL

SEQ ID NO: 11 - protein, 206 aa, Artificial Sequence
  source: /note="Description of Artificial Sequence: Synthetic polypeptide"
MVEEALNIFDECRSPCSLTPEPGKPIQSKLSIPSDVVLDEGVLYYSMTINDEQNDIKDEDKGESIITIGEFATVRATRHYVNQDAPFGVIHLDITTENGTKTYSYNRKEGEFAINWLVPIGEDSPASIKISVDELDQQRNIIEVPKLYSIDLDNQTLEQWKTQGNVSFSVTRPEHNIAISWPSVSYKAAQKEGSRHKRWAHWHTGL

SEQ ID NO: 12 - protein, 204 aa, Vibrio cholera
VEEALNIFDECRSPCSLTPEPGKPIQSKLSIPSDVVLDEGVLYYSMTINDEQNDIKDEDKGESIITIGEFATVRATRHYVNQDAPFGVIHLDITTENGTKTYSYNRKEGEFAINWLVPIGEDSPASIKISVDELDQQRNIIEVPKLYSIDLDNQTLEQWKTQGNVSFSVTRPEHNIAISWPSVSYKAAQKEGSRHKRWAHWHTG

SEQ ID NO: 13 - protein, 203 aa, Vibrio cholera
VEEALNIFDECRSPCSLTPEPGKPIQSKLSIPSDVVLDEGVLYYSMTINDEQNDIKDEDKGESIITIGEFATVRATRHYVNQDAPFGVIHLDITTENGTKTYSYNRKEGEFAINWLVPIGEDSPASIKISVDELDQQRNIIEVPKLYSIDLDNQTLEQWKTQGNVSFSVTRPEHNIAISWPSVSYKAAQKEGSRHKRWAHWHT

SEQ ID NO: 14 - protein, 202 aa, Vibrio cholera
VEEALNIFDECRSPCSLTPEPGKPIQSKLSIPSDVVLDEGVLYYSMTINDEQNDIKDEDKGESIITIGEFATVRATRHYVNQDAPFGVIHLDITTENGTKTYSYNRKEGEFAINWLVPIGEDSPASIKISVDELDQQRNIIEVPKLYSIDLDNQTLEQWKTQGNVSFSVTRPEHNIAISWPSVSYKAAQKEGSRHKRWAHWH

SEQ ID NO: 15 - protein, 201 aa, Vibrio cholera
VEEALNIFDECRSPCSLTPEPGKPIQSKLSIPSDVVLDEGVLYYSMTINDEQNDIKDEDKGESIITIGEFATVRATRHYVNQDAPFGVIHLDITTENGTKTYSYNRKEGEFAINWLVPIGEDSPASIKISVDELDQQRNIIEVPKLYSIDLDNQTLEQWKTQGNVSFSVTRPEHNIAISWPSVSYKAAQKEGSRHKRWAHW

SEQ ID NO: 16 - protein, 200 aa, Vibrio cholera
VEEALNIFDECRSPCSLTPEPGKPIQSKLSIPSDVVLDEGVLYYSMTINDEQNDIKDEDKGESIITIGEFATVRATRHYVNQDAPFGVIHLDITTENGTKTYSYNRKEGEFAINWLVPIGEDSPASIKISVDELDQQRNIIEVPKLYSIDLDNQTLEQWKTQGNVSFSVTRPEHNIAISWPSVSYKAAQKEGSRHKRWAH

SEQ ID NO: 17 - protein, 199 aa, Vibrio cholera
VEEALNIFDECRSPCSLTPEPGKPIQSKLSIPSDVVLDEGVLYYSMTINDEQNDIKDEDKGESIITIGEFATVRATRHYVNQDAPFGVIHLDITTENGTKTYSYNRKEGEFAINWLVPIGEDSPASIKISVDELDQQRNIIEVPKLYSIDLDNQTLEQWKTQGNVSFSVTRPEHNIAISWPSVSYKAAQKEGSRHKRWA

SEQ ID NO: 18 - protein, 198 aa, Vibrio cholera
VEEALNIFDECRSPCSLTPEPGKPIQSKLSIPSDVVLDEGVLYYSMTINDEQNDIKDEDKGESIITIGEFATVRATRHYVNQDAPFGVIHLDITTENGTKTYSYNRKEGEFAINWLVPIGEDSPASIKISVDELDQQRNIIEVPKLYSIDLDNQTLEQWKTQGNVSFSVTRPEHNIAISWPSVSYKAAQKEGSRHKRW

SEQ ID NO: 19 - protein, 197 aa, Vibrio cholera
VEEALNIFDECRSPCSLTPEPGKPIQSKLSIPSDVVLDEGVLYYSMTINDEQNDIKDEDKGESIITIGEFATVRATRHYVNQDAPFGVIHLDITTENGTKTYSYNRKEGEFAINWLVPIGEDSPASIKISVDELDQQRNIIEVPKLYSIDLDNQTLEQWKTQGNVSFSVTRPEHNIAISWPSVSYKAAQKEGSRHKR

SEQ ID NO: 20 - protein, 196 aa, Vibrio cholera
VEEALNIFDECRSPCSLTPEPGKPIQSKLSIPSDVVLDEGVLYYSMTINDEQNDIKDEDKGESIITIGEFATVRATRHYVNQDAPFGVIHLDITTENGTKTYSYNRKEGEFAINWLVPIGEDSPASIKISVDELDQQRNIIEVPKLYSIDLDNQTLEQWKTQGNVSFSVTRPEHNIAISWPSVSYKAAQKEGSRHK

SEQ ID NO: 21 - protein, 195 aa, Vibrio cholera
VEEALNIFDECRSPCSLTPEPGKPIQSKLSIPSDVVLDEGVLYYSMTINDEQNDIKDEDKGESIITIGEFATVRATRHYVNQDAPFGVIHLDITTENGTKTYSYNRKEGEFAINWLVPIGEDSPASIKISVDELDQQRNIIEVPKLYSIDLDNQTLEQWKTQGNVSFSVTRPEHNIAISWPSVSYKAAQKEGSRH

SEQ ID NO: 22 - protein, 194 aa, Vibrio cholera
VEEALNIFDECRSPCSLTPEPGKPIQSKLSIPSDVVLDEGVLYYSMTINDEQNDIKDEDKGESIITIGEFATVRATRHYVNQDAPFGVIHLDITTENGTKTYSYNRKEGEFAINWLVPIGEDSPASIKISVDELDQQRNIIEVPKLYSIDLDNQTLEQWKTQGNVSFSVTRPEHNIAISWPSVSYKAAQKEGSR

SEQ ID NO: 23 - protein, 193 aa, Vibrio cholera
VEEALNIFDECRSPCSLTPEPGKPIQSKLSIPSDVVLDEGVLYYSMTINDEQNDIKDEDKGESIITIGEFATVRATRHYVNQDAPFGVIHLDITTENGTKTYSYNRKEGEFAINWLVPIGEDSPASIKISVDELDQQRNIIEVPKLYSIDLDNQTLEQWKTQGNVSFSVTRPEHNIAISWPSVSYKAAQKEGS

SEQ ID NO: 24 - protein, 192 aa, Vibrio cholera
VEEALNIFDECRSPCSLTPEPGKPIQSKLSIPSDVVLDEGVLYYSMTINDEQNDIKDEDKGESIITIGEFATVRATRHYVNQDAPFGVIHLDITTENGTKTYSYNRKEGEFAINWLVPIGEDSPASIKISVDELDQQRNIIEVPKLYSIDLDNQTLEQWKTQGNVSFSVTRPEHNIAISWPSVSYKAAQKEG

SEQ ID NO: 25 - protein, 191 aa, Vibrio cholera
VEEALNIFDECRSPCSLTPEPGKPIQSKLSIPSDVVLDEGVLYYSMTINDEQNDIKDEDKGESIITIGEFATVRATRHYVNQDAPFGVIHLDITTENGTKTYSYNRKEGEFAINWLVPIGEDSPASIKISVDELDQQRNIIEVPKLYSIDLDNQTLEQWKTQGNVSFSVTRPEHNIAISWPSVSYKAAQKE

SEQ ID NO: 26 - protein, 190 aa, Vibrio cholera
VEEALNIFDECRSPCSLTPEPGKPIQSKLSIPSDVVLDEGVLYYSMTINDEQNDIKDEDKGESIITIGEFATVRATRHYVNQDAPFGVIHLDITTENGTKTYSYNRKEGEFAINWLVPIGEDSPASIKISVDELDQQRNIIEVPKLYSIDLDNQTLEQWKTQGNVSFSVTRPEHNIAISWPSVSYKAAQK

SEQ ID NO: 27 - protein, 189 aa, Vibrio cholera
VEEALNIFDECRSPCSLTPEPGKPIQSKLSIPSDVVLDEGVLYYSMTINDEQNDIKDEDKGESIITIGEFATVRATRHYVNQDAPFGVIHLDITTENGTKTYSYNRKEGEFAINWLVPIGEDSPASIKISVDELDQQRNIIEVPKLYSIDLDNQTLEQWKTQGNVSFSVTRPEHNIAISWPSVSYKAAQ

SEQ ID NO: 28 - protein, 188 aa, Vibrio cholera
VEEALNIFDECRSPCSLTPEPGKPIQSKLSIPSDVVLDEGVLYYSMTINDEQNDIKDEDKGESIITIGEFATVRATRHYVNQDAPFGVIHLDITTENGTKTYSYNRKEGEFAINWLVPIGEDSPASIKISVDELDQQRNIIEVPKLYSIDLDNQTLEQWKTQGNVSFSVTRPEHNIAISWPSVSYKAA

SEQ ID NO: 29 - protein, 187 aa, Vibrio cholera
VEEALNIFDECRSPCSLTPEPGKPIQSKLSIPSDVVLDEGVLYYSMTINDEQNDIKDEDKGESIITIGEFATVRATRHYVNQDAPFGVIHLDITTENGTKTYSYNRKEGEFAINWLVPIGEDSPASIKISVDELDQQRNIIEVPKLYSIDLDNQTLEQWKTQGNVSFSVTRPEHNIAISWPSVSYKA

SEQ ID NO: 30 - protein, 186 aa, Vibrio cholera
VEEALNIFDECRSPCSLTPEPGKPIQSKLSIPSDVVLDEGVLYYSMTINDEQNDIKDEDKGESIITIGEFATVRATRHYVNQDAPFGVIHLDITTENGTKTYSYNRKEGEFAINWLVPIGEDSPASIKISVDELDQQRNIIEVPKLYSIDLDNQTLEQWKTQGNVSFSVTRPEHNIAISWPSVSYK

SEQ ID NO: 31 - protein, 187 aa, Artificial Sequence
  source: /note="Description of Artificial Sequence: Synthetic polypeptide"
MVEEALNIFDECRSPCSLTPEPGKPIQSKLSIPSDVVLDEGVLYYSMTINDEQNDIKDEDKGESIITIGEFATVRATRHYVNQDAPFGVIHLDITTENGTKTYSYNRKEGEFAINWLVPIGEDSPASIKISVDELDQQRNIIEVPKLYSIDLDNQTLEQWKTQGNVSFSVTRPEHNIAISWPSVSYK

SEQ ID NO: 32 - protein, 185 aa, Vibrio cholera
EEALNIFDECRSPCSLTPEPGKPIQSKLSIPSDVVLDEGVLYYSMTINDEQNDIKDEDKGESIITIGEFATVRATRHYVNQDAPFGVIHLDITTENGTKTYSYNRKEGEFAINWLVPIGEDSPASIKISVDELDQQRNIIEVPKLYSIDLDNQTLEQWKTQGNVSFSVTRPEHNIAISWPSVSYK

SEQ ID NO: 33 - protein, 184 aa, Vibrio cholera
EALNIFDECRSPCSLTPEPGKPIQSKLSIPSDVVLDEGVLYYSMTINDEQNDIKDEDKGESIITIGEFATVRATRHYVNQDAPFGVIHLDITTENGTKTYSYNRKEGEFAINWLVPIGEDSPASIKISVDELDQQRNIIEVPKLYSIDLDNQTLEQWKTQGNVSFSVTRPEHNIAISWPSVSYK

SEQ ID NO: 34 - protein, 183 aa, Vibrio cholera
ALNIFDECRSPCSLTPEPGKPIQSKLSIPSDVVLDEGVLYYSMTINDEQNDIKDEDKGESIITIGEFATVRATRHYVNQDAPFGVIHLDITTENGTKTYSYNRKEGEFAINWLVPIGEDSPASIKISVDELDQQRNIIEVPKLYSIDLDNQTLEQWKTQGNVSFSVTRPEHNIAISWPSVSYK

SEQ ID NO: 35 - protein, 182 aa, Vibrio cholera
LNIFDECRSPCSLTPEPGKPIQSKLSIPSDVVLDEGVLYYSMTINDEQNDIKDEDKGESIITIGEFATVRATRHYVNQDAPFGVIHLDITTENGTKTYSYNRKEGEFAINWLVPIGEDSPASIKISVDELDQQRNIIEVPKLYSIDLDNQTLEQWKTQGNVSFSVTRPEHNIAISWPSVSYK

SEQ ID NO: 36 - protein, 181 aa, Vibrio cholera
NIFDECRSPCSLTPEPGKPIQSKLSIPSDVVLDEGVLYYSMTINDEQNDIKDEDKGESIITIGEFATVRATRHYVNQDAPFGVIHLDITTENGTKTYSYNRKEGEFAINWLVPIGEDSPASIKISVDELDQQRNIIEVPKLYSIDLDNQTLEQWKTQGNVSFSVTRPEHNIAISWPSVSYK

SEQ ID NO: 37 - protein, 180 aa, Vibrio cholera
IFDECRSPCSLTPEPGKPIQSKLSIPSDVVLDEGVLYYSMTINDEQNDIKDEDKGESIITIGEFATVRATRHYVNQDAPFGVIHLDITTENGTKTYSYNRKEGEFAINWLVPIGEDSPASIKISVDELDQQRNIIEVPKLYSIDLDNQTLEQWKTQGNVSFSVTRPEHNIAISWPSVSYK

SEQ ID NO: 38 - protein, 179 aa, Vibrio cholera
FDECRSPCSLTPEPGKPIQSKLSIPSDVVLDEGVLYYSMTINDEQNDIKDEDKGESIITIGEFATVRATRHYVNQDAPFGVIHLDITTENGTKTYSYNRKEGEFAINWLVPIGEDSPASIKISVDELDQQRNIIEVPKLYSIDLDNQTLEQWKTQGNVSFSVTRPEHNIAISWPSVSYK

SEQ ID NO: 39 - protein, 178 aa, Vibrio cholera
DECRSPCSLTPEPGKPIQSKLSIPSDVVLDEGVLYYSMTINDEQNDIKDEDKGESIITIGEFATVRATRHYVNQDAPFGVIHLDITTENGTKTYSYNRKEGEFAINWLVPIGEDSPASIKISVDELDQQRNIIEVPKLYSIDLDNQTLEQWKTQGNVSFSVTRPEHNIAISWPSVSYK

SEQ ID NO: 40 - protein, 177 aa, Vibrio cholera
ECRSPCSLTPEPGKPIQSKLSIPSDVVLDEGVLYYSMTINDEQNDIKDEDKGESIITIGEFATVRATRHYVNQDAPFGVIHLDITTENGTKTYSYNRKEGEFAINWLVPIGEDSPASIKISVDELDQQRNIIEVPKLYSIDLDNQTLEQWKTQGNVSFSVTRPEHNIAISWPSVSYK

SEQ ID NO: 41 - protein, 176 aa, Vibrio cholera
CRSPCSLTPEPGKPIQSKLSIPSDVVLDEGVLYYSMTINDEQNDIKDEDKGESIITIGEFATVRATRHYVNQDAPFGVIHLDITTENGTKTYSYNRKEGEFAINWLVPIGEDSPASIKISVDELDQQRNIIEVPKLYSIDLDNQTLEQWKTQGNVSFSVTRPEHNIAISWPSVSYK

SEQ ID NO: 42 - protein, 175 aa, Vibrio cholera
RSPCSLTPEPGKPIQSKLSIPSDVVLDEGVLYYSMTINDEQNDIKDEDKGESIITIGEFATVRATRHYVNQDAPFGVIHLDITTENGTKTYSYNRKEGEFAINWLVPIGEDSPASIKISVDELDQQRNIIEVPKLYSIDLDNQTLEQWKTQGNVSFSVTRPEHNIAISWPSVSYK

SEQ ID NO: 43 - protein, 174 aa, Vibrio cholera
SPCSLTPEPGKPIQSKLSIPSDVVLDEGVLYYSMTINDEQNDIKDEDKGESIITIGEFATVRATRHYVNQDAPFGVIHLDITTENGTKTYSYNRKEGEFAINWLVPIGEDSPASIKISVDELDQQRNIIEVPKLYSIDLDNQTLEQWKTQGNVSFSVTRPEHNIAISWPSVSYK

SEQ ID NO: 44 - protein, 173 aa, Vibrio cholera
PCSLTPEPGKPIQSKLSIPSDVVLDEGVLYYSMTINDEQNDIKDEDKGESIITIGEFATVRATRHYVNQDAPFGVIHLDITTENGTKTYSYNRKEGEFAINWLVPIGEDSPASIKISVDELDQQRNIIEVPKLYSIDLDNQTLEQWKTQGNVSFSVTRPEHNIAISWPSVSYK

SEQ ID NO: 45 - protein, 172 aa, Vibrio cholera
CSLTPEPGKPIQSKLSIPSDVVLDEGVLYYSMTINDEQNDIKDEDKGESIITIGEFATVRATRHYVNQDAPFGVIHLDITTENGTKTYSYNRKEGEFAINWLVPIGEDSPASIKISVDELDQQRNIIEVPKLYSIDLDNQTLEQWKTQGNVSFSVTRPEHNIAISWPSVSYK

SEQ ID NO: 46 - protein, 171 aa, Vibrio cholera
SLTPEPGKPIQSKLSIPSDVVLDEGVLYYSMTINDEQNDIKDEDKGESIITIGEFATVRATRHYVNQDAPFGVIHLDITTENGTKTYSYNRKEGEFAINWLVPIGEDSPASIKISVDELDQQRNIIEVPKLYSIDLDNQTLEQWKTQGNVSFSVTRPEHNIAISWPSVSYK

SEQ ID NO: 47 - protein, 170 aa, Vibrio cholera
LTPEPGKPIQSKLSIPSDVVLDEGVLYYSMTINDEQNDIKDEDKGESIITIGEFATVRATRHYVNQDAPFGVIHLDITTENGTKTYSYNRKEGEFAINWLVPIGEDSPASIKISVDELDQQRNIIEVPKLYSIDLDNQTLEQWKTQGNVSFSVTRPEHNIAISWPSVSYK

SEQ ID NO: 48 - protein, 169 aa, Vibrio cholera
TPEPGKPIQSKLSIPSDVVLDEGVLYYSMTINDEQNDIKDEDKGESIITIGEFATVRATRHYVNQDAPFGVIHLDITTENGTKTYSYNRKEGEFAINWLVPIGEDSPASIKISVDELDQQRNIIEVPKLYSIDLDNQTLEQWKTQGNVSFSVTRPEHNIAISWPSVSYK

SEQ ID NO: 49 - protein, 168 aa, Vibrio cholera
PEPGKPIQSKLSIPSDVVLDEGVLYYSMTINDEQNDIKDEDKGESIITIGEFATVRATRHYVNQDAPFGVIHLDITTENGTKTYSYNRKEGEFAINWLVPIGEDSPASIKISVDELDQQRNIIEVPKLYSIDLDNQTLEQWKTQGNVSFSVTRPEHNIAISWPSVSYK

SEQ ID NO: 50 - protein, 167 aa, Vibrio cholera
EPGKPIQSKLSIPSDVVLDEGVLYYSMTINDEQNDIKDEDKGESIITIGEFATVRATRHYVNQDAPFGVIHLDITTENGTKTYSYNRKEGEFAINWLVPIGEDSPASIKISVDELDQQRNIIEVPKLYSIDLDNQTLEQWKTQGNVSFSVTRPEHNIAISWPSVSYK

SEQ ID NO: 51 - protein, 166 aa, Vibrio cholera
PGKPIQSKLSIPSDVVLDEGVLYYSMTINDEQNDIKDEDKGESIITIGEFATVRATRHYVNQDAPFGVIHLDITTENGTKTYSYNRKEGEFAINWLVPIGEDSPASIKISVDELDQQRNIIEVPKLYSIDLDNQTLEQWKTQGNVSFSVTRPEHNIAISWPSVSYK

SEQ ID NO: 52 - protein, 165 aa, Vibrio cholera
GKPIQSKLSIPSDVVLDEGVLYYSMTINDEQNDIKDEDKGESIITIGEFATVRATRHYVNQDAPFGVIHLDITTENGTKTYSYNRKEGEFAINWLVPIGEDSPASIKISVDELDQQRNIIEVPKLYSIDLDNQTLEQWKTQGNVSFSVTRPEHNIAISWPSVSYK

SEQ ID NO: 53 - protein, 164 aa, Vibrio cholera
KPIQSKLSIPSDVVLDEGVLYYSMTINDEQNDIKDEDKGESIITIGEFATVRATRHYVNQDAPFGVIHLDITTENGTKTYSYNRKEGEFAINWLVPIGEDSPASIKISVDELDQQRNIIEVPKLYSIDLDNQTLEQWKTQGNVSFSVTRPEHNIAISWPSVSYK

SEQ ID NO: 54 - protein, 163 aa, Vibrio cholera
PIQSKLSIPSDVVLDEGVLYYSMTINDEQNDIKDEDKGESIITIGEFATVRATRHYVNQDAPFGVIHLDITTENGTKTYSYNRKEGEFAINWLVPIGEDSPASIKISVDELDQQRNIIEVPKLYSIDLDNQTLEQWKTQGNVSFSVTRPEHNIAISWPSVSYK

SEQ ID NO: 55 - protein, 162 aa, Vibrio cholera
IQSKLSIPSDVVLDEGVLYYSMTINDEQNDIKDEDKGESIITIGEFATVRATRHYVNQDAPFGVIHLDITTENGTKTYSYNRKEGEFAINWLVPIGEDSPASIKISVDELDQQRNIIEVPKLYSIDLDNQTLEQWKTQGNVSFSVTRPEHNIAISWPSVSYK

SEQ ID NO: 56 - protein, 161 aa, Vibrio cholera
QSKLSIPSDVVLDEGVLYYSMTINDEQNDIKDEDKGESIITIGEFATVRATRHYVNQDAPFGVIHLDITTENGTKTYSYNRKEGEFAINWLVPIGEDSPASIKISVDELDQQRNIIEVPKLYSIDLDNQTLEQWKTQGNVSFSVTRPEHNIAISWPSVSYK

SEQ ID NO: 57 - protein, 160 aa, Vibrio cholera
SKLSIPSDVVLDEGVLYYSMTINDEQNDIKDEDKGESIITIGEFATVRATRHYVNQDAPFGVIHLDITTENGTKTYSYNRKEGEFAINWLVPIGEDSPASIKISVDELDQQRNIIEVPKLYSIDLDNQTLEQWKTQGNVSFSVTRPEHNIAISWPSVSYK

SEQ ID NO: 58 - protein, 159 aa, Vibrio cholera
KLSIPSDVVLDEGVLYYSMTINDEQNDIKDEDKGESIITIGEFATVRATRHYVNQDAPFGVIHLDITTENGTKTYSYNRKEGEFAINWLVPIGEDSPASIKISVDELDQQRNIIEVPKLYSIDLDNQTLEQWKTQGNVSFSVTRPEHNIAISWPSVSYK

SEQ ID NO: 59 - protein, 158 aa, Vibrio cholera
LSIPSDVVLDEGVLYYSMTINDEQNDIKDEDKGESIITIGEFATVRATRHYVNQDAPFGVIHLDITTENGTKTYSYNRKEGEFAINWLVPIGEDSPASIKISVDELDQQRNIIEVPKLYSIDLDNQTLEQWKTQGNVSFSVTRPEHNIAISWPSVSYK

SEQ ID NO: 60 - protein, 157 aa, Vibrio cholera
SIPSDVVLDEGVLYYSMTINDEQNDIKDEDKGESIITIGEFATVRATRHYVNQDAPFGVIHLDITTENGTKTYSYNRKEGEFAINWLVPIGEDSPASIKISVDELDQQRNIIEVPKLYSIDLDNQTLEQWKTQGNVSFSVTRPEHNIAISWPSVSYK

SEQ ID NO: 61 - protein, 156 aa, Vibrio cholera
IPSDVVLDEGVLYYSMTINDEQNDIKDEDKGESIITIGEFATVRATRHYVNQDAPFGVIHLDITTENGTKTYSYNRKEGEFAINWLVPIGEDSPASIKISVDELDQQRNIIEVPKLYSIDLDNQTLEQWKTQGNVSFSVTRPEHNIAISWPSVSYK

SEQ ID NO: 62 - protein, 155 aa, Vibrio cholera
PSDVVLDEGVLYYSMTINDEQNDIKDEDKGESIITIGEFATVRATRHYVNQDAPFGVIHLDITTENGTKTYSYNRKEGEFAINWLVPIGEDSPASIKISVDELDQQRNIIEVPKLYSIDLDNQTLEQWKTQGNVSFSVTRPEHNIAISWPSVSYK

SEQ ID NO: 63 - protein, 154 aa, Vibrio cholera
SDVVLDEGVLYYSMTINDEQNDIKDEDKGESIITIGEFATVRATRHYVNQDAPFGVIHLDITTENGTKTYSYNRKEGEFAINWLVPIGEDSPASIKISVDELDQQRNIIEVPKLYSIDLDNQTLEQWKTQGNVSFSVTRPEHNIAISWPSVSYK

SEQ ID NO: 64 - protein, 153 aa, Vibrio cholera
DVVLDEGVLYYSMTINDEQNDIKDEDKGESIITIGEFATVRATRHYVNQDAPFGVIHLDITTENGTKTYSYNRKEGEFAINWLVPIGEDSPASIKISVDELDQQRNIIEVPKLYSIDLDNQTLEQWKTQGNVSFSVTRPEHNIAISWPSVSYK

SEQ ID NO: 65 - protein, 152 aa, Vibrio cholera
VVLDEGVLYYSMTINDEQNDIKDEDKGESIITIGEFATVRATRHYVNQDAPFGVIHLDITTENGTKTYSYNRKEGEFAINWLVPIGEDSPASIKISVDELDQQRNIIEVPKLYSIDLDNQTLEQWKTQGNVSFSVTRPEHNIAISWPSVSYK

SEQ ID NO: 66 - protein, 151 aa, Vibrio cholera
VLDEGVLYYSMTINDEQNDIKDEDKGESIITIGEFATVRATRHYVNQDAPFGVIHLDITTENGTKTYSYNRKEGEFAINWLVPIGEDSPASIKISVDELDQQRNIIEVPKLYSIDLDNQTLEQWKTQGNVSFSVTRPEHNIAISWPSVSYK

SEQ ID NO: 67 - protein, 150 aa, Vibrio cholera
LDEGVLYYSMTINDEQNDIKDEDKGESIITIGEFATVRATRHYVNQDAPFGVIHLDITTENGTKTYSYNRKEGEFAINWLVPIGEDSPASIKISVDELDQQRNIIEVPKLYSIDLDNQTLEQWKTQGNVSFSVTRPEHNIAISWPSVSYK

SEQ ID NO: 68 - protein, 149 aa, Vibrio cholera
DEGVLYYSMTINDEQNDIKDEDKGESIITIGEFATVRATRHYVNQDAPFGVIHLDITTENGTKTYSYNRKEGEFAINWLVPIGEDSPASIKISVDELDQQRNIIEVPKLYSIDLDNQTLEQWKTQGNVSFSVTRPEHNIAISWPSVSYK

SEQ ID NO: 69 - protein, 148 aa, Vibrio cholera
EGVLYYSMTINDEQNDIKDEDKGESIITIGEFATVRATRHYVNQDAPFGVIHLDITTENGTKTYSYNRKEGEFAINWLVPIGEDSPASIKISVDELDQQRNIIEVPKLYSIDLDNQTLEQWKTQGNVSFSVTRPEHNIAISWPSVSYK

SEQ ID NO: 70 - protein, 147 aa, Vibrio cholera
GVLYYSMTINDEQNDIKDEDKGESIITIGEFATVRATRHYVNQDAPFGVIHLDITTENGTKTYSYNRKEGEFAINWLVPIGEDSPASIKISVDELDQQRNIIEVPKLYSIDLDNQTLEQWKTQGNVSFSVTRPEHNIAISWPSVSYK

SEQ ID NO: 71 - protein, 185 aa, Vibrio cholera
VEEALNIFDECRSPCSLTPEPGKPIQSKLSIPSDVVLDEGVLYYSMTINDEQNDIKDEDKGESIITIGEFATVRATRHYVNQDAPFGVIHLDITTENGTKTYSYNRKEGEFAINWLVPIGEDSPASIKISVDELDQQRNIIEVPKLYSIDLDNQTLEQWKTQGNVSFSVTRPEHNIAISWPSVSY

SEQ ID NO: 72 - protein, 184 aa, Vibrio cholera
VEEALNIFDECRSPCSLTPEPGKPIQSKLSIPSDVVLDEGVLYYSMTINDEQNDIKDEDKGESIITIGEFATVRATRHYVNQDAPFGVIHLDITTENGTKTYSYNRKEGEFAINWLVPIGEDSPASIKISVDELDQQRNIIEVPKLYSIDLDNQTLEQWKTQGNVSFSVTRPEHNIAISWPSVS

SEQ ID NO: 73 - protein, 183 aa, Vibrio cholera
VEEALNIFDECRSPCSLTPEPGKPIQSKLSIPSDVVLDEGVLYYSMTINDEQNDIKDEDKGESIITIGEFATVRATRHYVNQDAPFGVIHLDITTENGTKTYSYNRKEGEFAINWLVPIGEDSPASIKISVDELDQQRNIIEVPKLYSIDLDNQTLEQWKTQGNVSFSVTRPEHNIAISWPSV

SEQ ID NO: 74 - protein, 182 aa, Vibrio cholera
VEEALNIFDECRSPCSLTPEPGKPIQSKLSIPSDVVLDEGVLYYSMTINDEQNDIKDEDKGESIITIGEFATVRATRHYVNQDAPFGVIHLDITTENGTKTYSYNRKEGEFAINWLVPIGEDSPASIKISVDELDQQRNIIEVPKLYSIDLDNQTLEQWKTQGNVSFSVTRPEHNIAISWPS

SEQ ID NO: 75 - protein, 181 aa, Vibrio cholera
VEEALNIFDECRSPCSLTPEPGKPIQSKLSIPSDVVLDEGVLYYSMTINDEQNDIKDEDKGESIITIGEFATVRATRHYVNQDAPFGVIHLDITTENGTKTYSYNRKEGEFAINWLVPIGEDSPASIKISVDELDQQRNIIEVPKLYSIDLDNQTLEQWKTQGNVSFSVTRPEHNIAISWP

SEQ ID NO: 76 - protein, 180 aa, Vibrio cholera
VEEALNIFDECRSPCSLTPEPGKPIQSKLSIPSDVVLDEGVLYYSMTINDEQNDIKDEDKGESIITIGEFATVRATRHYVNQDAPFGVIHLDITTENGTKTYSYNRKEGEFAINWLVPIGEDSPASIKISVDELDQQRNIIEVPKLYSIDLDNQTLEQWKTQGNVSFSVTRPEHNIAISW

SEQ ID NO: 77 - protein, 179 aa, Vibrio cholera
VEEALNIFDECRSPCSLTPEPGKPIQSKLSIPSDVVLDEGVLYYSMTINDEQNDIKDEDKGESIITIGEFATVRATRHYVNQDAPFGVIHLDITTENGTKTYSYNRKEGEFAINWLVPIGEDSPASIKISVDELDQQRNIIEVPKLYSIDLDNQTLEQWKTQGNVSFSVTRPEHNIAIS

SEQ ID NO: 78 - protein, 178 aa, Vibrio cholera
VEEALNIFDECRSPCSLTPEPGKPIQSKLSIPSDVVLDEGVLYYSMTINDEQNDIKDEDKGESIITIGEFATVRATRHYVNQDAPFGVIHLDITTENGTKTYSYNRKEGEFAINWLVPIGEDSPASIKISVDELDQQRNIIEVPKLYSIDLDNQTLEQWKTQGNVSFSVTRPEHNIAI

SEQ ID NO: 79 - protein, 177 aa, Vibrio cholera
VEEALNIFDECRSPCSLTPEPGKPIQSKLSIPSDVVLDEGVLYYSMTINDEQNDIKDEDKGESIITIGEFATVRATRHYVNQDAPFGVIHLDITTENGTKTYSYNRKEGEFAINWLVPIGEDSPASIKISVDELDQQRNIIEVPKLYSIDLDNQTLEQWKTQGNVSFSVTRPEHNIA

SEQ ID NO: 80 - protein, 176 aa, Vibrio cholera
VEEALNIFDECRSPCSLTPEPGKPIQSKLSIPSDVVLDEGVLYYSMTINDEQNDIKDEDKGESIITIGEFATVRATRHYVNQDAPFGVIHLDITTENGTKTYSYNRKEGEFAINWLVPIGEDSPASIKISVDELDQQRNIIEVPKLYSIDLDNQTLEQWKTQGNVSFSVTRPEHNI

SEQ ID NO: 81 - protein, 175 aa, Vibrio cholera
VEEALNIFDECRSPCSLTPEPGKPIQSKLSIPSDVVLDEGVLYYSMTINDEQNDIKDEDKGESIITIGEFATVRATRHYVNQDAPFGVIHLDITTENGTKTYSYNRKEGEFAINWLVPIGEDSPASIKISVDELDQQRNIIEVPKLYSIDLDNQTLEQWKTQGNVSFSVTRPEHN

SEQ ID NO: 82 - protein, 174 aa, Vibrio cholera
VEEALNIFDECRSPCSLTPEPGKPIQSKLSIPSDVVLDEGVLYYSMTINDEQNDIKDEDKGESIITIGEFATVRATRHYVNQDAPFGVIHLDITTENGTKTYSYNRKEGEFAINWLVPIGEDSPASIKISVDELDQQRNIIEVPKLYSIDLDNQTLEQWKTQGNVSFSVTRPEH

SEQ ID NO: 83 - protein, 173 aa, Vibrio cholera
VEEALNIFDECRSPCSLTPEPGKPIQSKLSIPSDVVLDEGVLYYSMTINDEQNDIKDEDKGESIITIGEFATVRATRHYVNQDAPFGVIHLDITTENGTKTYSYNRKEGEFAINWLVPIGEDSPASIKISVDELDQQRNIIEVPKLYSIDLDNQTLEQWKTQGNVSFSVTRPE

SEQ ID NO: 84 - protein, 172 aa, Vibrio cholera
VEEALNIFDECRSPCSLTPEPGKPIQSKLSIPSDVVLDEGVLYYSMTINDEQNDIKDEDKGESIITIGEFATVRATRHYVNQDAPFGVIHLDITTENGTKTYSYNRKEGEFAINWLVPIGEDSPASIKISVDELDQQRNIIEVPKLYSIDLDNQTLEQWKTQGNVSFSVTRP

SEQ ID NO: 85 - protein, 171 aa, Vibrio cholera
VEEALNIFDECRSPCSLTPEPGKPIQSKLSIPSDVVLDEGVLYYSMTINDEQNDIKDEDKGESIITIGEFATVRATRHYVNQDAPFGVIHLDITTENGTKTYSYNRKEGEFAINWLVPIGEDSPASIKISVDELDQQRNIIEVPKLYSIDLDNQTLEQWKTQGNVSFSVTR

SEQ ID NO: 86 - protein, 170 aa, Vibrio cholera
VEEALNIFDECRSPCSLTPEPGKPIQSKLSIPSDVVLDEGVLYYSMTINDEQNDIKDEDKGESIITIGEFATVRATRHYVNQDAPFGVIHLDITTENGTKTYSYNRKEGEFAINWLVPIGEDSPASIKISVDELDQQRNIIEVPKLYSIDLDNQTLEQWKTQGNVSFSVT

SEQ ID NO: 87 - protein, 169 aa, Vibrio cholera
VEEALNIFDECRSPCSLTPEPGKPIQSKLSIPSDVVLDEGVLYYSMTINDEQNDIKDEDKGESIITIGEFATVRATRHYVNQDAPFGVIHLDITTENGTKTYSYNRKEGEFAINWLVPIGEDSPASIKISVDELDQQRNIIEVPKLYSIDLDNQTLEQWKTQGNVSFSV

SEQ ID NO: 88 - protein, 168 aa, Vibrio cholera
VEEALNIFDECRSPCSLTPEPGKPIQSKLSIPSDVVLDEGVLYYSMTINDEQNDIKDEDKGESIITIGEFATVRATRHYVNQDAPFGVIHLDITTENGTKTYSYNRKEGEFAINWLVPIGEDSPASIKISVDELDQQRNIIEVPKLYSIDLDNQTLEQWKTQGNVSFS

SEQ ID NO: 89 - protein, 167 aa, Vibrio cholera
VEEALNIFDECRSPCSLTPEPGKPIQSKLSIPSDVVLDEGVLYYSMTINDEQNDIKDEDKGESIITIGEFATVRATRHYVNQDAPFGVIHLDITTENGTKTYSYNRKEGEFAINWLVPIGEDSPASIKISVDELDQQRNIIEVPKLYSIDLDNQTLEQWKTQGNVSF

SEQ ID NO: 90 - protein, 166 aa, Vibrio cholera
VEEALNIFDECRSPCSLTPEPGKPIQSKLSIPSDVVLDEGVLYYSMTINDEQNDIKDEDKGESIITIGEFATVRATRHYVNQDAPFGVIHLDITTENGTKTYSYNRKEGEFAINWLVPIGEDSPASIKISVDELDQQRNIIEVPKLYSIDLDNQTLEQWKTQGNVS

SEQ ID NO: 91 - protein, 165 aa, Vibrio cholera
VEEALNIFDECRSPCSLTPEPGKPIQSKLSIPSDVVLDEGVLYYSMTINDEQNDIKDEDKGESIITIGEFATVRATRHYVNQDAPFGVIHLDITTENGTKTYSYNRKEGEFAINWLVPIGEDSPASIKISVDELDQQRNIIEVPKLYSIDLDNQTLEQWKTQGNV

SEQ ID NO: 92 - protein, 164 aa, Vibrio cholera
VEEALNIFDECRSPCSLTPEPGKPIQSKLSIPSDVVLDEGVLYYSMTINDEQNDIKDEDKGESIITIGEFATVRATRHYVNQDAPFGVIHLDITTENGTKTYSYNRKEGEFAINWLVPIGEDSPASIKISVDELDQQRNIIEVPKLYSIDLDNQTLEQWKTQGN

SEQ ID NO: 93 - protein, 163 aa, Vibrio cholera
VEEALNIFDECRSPCSLTPEPGKPIQSKLSIPSDVVLDEGVLYYSMTINDEQNDIKDEDKGESIITIGEFATVRATRHYVNQDAPFGVIHLDITTENGTKTYSYNRKEGEFAINWLVPIGEDSPASIKISVDELDQQRNIIEVPKLYSIDLDNQTLEQWKTQG

SEQ ID NO: 94 - protein, 162 aa, Vibrio cholera
VEEALNIFDECRSPCSLTPEPGKPIQSKLSIPSDVVLDEGVLYYSMTINDEQNDIKDEDKGESIITIGEFATVRATRHYVNQDAPFGVIHLDITTENGTKTYSYNRKEGEFAINWLVPIGEDSPASIKISVDELDQQRNIIEVPKLYSIDLDNQTLEQWKTQ

SEQ ID NO: 95 - protein, 161 aa, Vibrio cholera
VEEALNIFDECRSPCSLTPEPGKPIQSKLSIPSDVVLDEGVLYYSMTINDEQNDIKDEDKGESIITIGEFATVRATRHYVNQDAPFGVIHLDITTENGTKTYSYNRKEGEFAINWLVPIGEDSPASIKISVDELDQQRNIIEVPKLYSIDLDNQTLEQWKT

SEQ ID NO: 96 - protein, 160 aa, Vibrio cholera
VEEALNIFDECRSPCSLTPEPGKPIQSKLSIPSDVVLDEGVLYYSMTINDEQNDIKDEDKGESIITIGEFATVRATRHYVNQDAPFGVIHLDITTENGTKTYSYNRKEGEFAINWLVPIGEDSPASIKISVDELDQQRNIIEVPKLYSIDLDNQTLEQWK

SEQ ID NO: 97 - protein, 159 aa, Vibrio cholera
VEEALNIFDECRSPCSLTPEPGKPIQSKLSIPSDVVLDEGVLYYSMTINDEQNDIKDEDKGESIITIGEFATVRATRHYVNQDAPFGVIHLDITTENGTKTYSYNRKEGEFAINWLVPIGEDSPASIKISVDELDQQRNIIEVPKLYSIDLDNQTLEQW

SEQ ID NO: 98 - protein, 158 aa, Vibrio cholera
VEEALNIFDECRSPCSLTPEPGKPIQSKLSIPSDVVLDEGVLYYSMTINDEQNDIKDEDKGESIITIGEFATVRATRHYVNQDAPFGVIHLDITTENGTKTYSYNRKEGEFAINWLVPIGEDSPASIKISVDELDQQRNIIEVPKLYSIDLDNQTLEQ

SEQ ID NO: 99 - protein, 157 aa, Vibrio cholera
VEEALNIFDECRSPCSLTPEPGKPIQSKLSIPSDVVLDEGVLYYSMTINDEQNDIKDEDKGESIITIGEFATVRATRHYVNQDAPFGVIHLDITTENGTKTYSYNRKEGEFAINWLVPIGEDSPASIKISVDELDQQRNIIEVPKLYSIDLDNQTLE

SEQ ID NO: 100 - protein, 156 aa, Vibrio cholera
VEEALNIFDECRSPCSLTPEPGKPIQSKLSIPSDVVLDEGVLYYSMTINDEQNDIKDEDKGESIITIGEFATVRATRHYVNQDAPFGVIHLDITTENGTKTYSYNRKEGEFAINWLVPIGEDSPASIKISVDELDQQRNIIEVPKLYSIDLDNQTL

SEQ ID NO: 101 - protein, 155 aa, Vibrio cholera
VEEALNIFDECRSPCSLTPEPGKPIQSKLSIPSDVVLDEGVLYYSMTINDEQNDIKDEDKGESIITIGEFATVRATRHYVNQDAPFGVIHLDITTENGTKTYSYNRKEGEFAINWLVPIGEDSPASIKISVDELDQQRNIIEVPKLYSIDLDNQT

SEQ ID NO: 102 - protein, 154 aa, Vibrio cholera
VEEALNIFDECRSPCSLTPEPGKPIQSKLSIPSDVVLDEGVLYYSMTINDEQNDIKDEDKGESIITIGEFATVRATRHYVNQDAPFGVIHLDITTENGTKTYSYNRKEGEFAINWLVPIGEDSPASIKISVDELDQQRNIIEVPKLYSIDLDNQ

SEQ ID NO: 103 - protein, 153 aa, Vibrio cholera
VEEALNIFDECRSPCSLTPEPGKPIQSKLSIPSDVVLDEGVLYYSMTINDEQNDIKDEDKGESIITIGEFATVRATRHYVNQDAPFGVIHLDITTENGTKTYSYNRKEGEFAINWLVPIGEDSPASIKISVDELDQQRNIIEVPKLYSIDLDN

SEQ ID NO: 104 - protein, 152 aa, Vibrio cholera
VEEALNIFDECRSPCSLTPEPGKPIQSKLSIPSDVVLDEGVLYYSMTINDEQNDIKDEDKGESIITIGEFATVRATRHYVNQDAPFGVIHLDITTENGTKTYSYNRKEGEFAINWLVPIGEDSPASIKISVDELDQQRNIIEVPKLYSIDLD

SEQ ID NO: 105 - protein, 151 aa, Vibrio cholera
VEEALNIFDECRSPCSLTPEPGKPIQSKLSIPSDVVLDEGVLYYSMTINDEQNDIKDEDKGESIITIGEFATVRATRHYVNQDAPFGVIHLDITTENGTKTYSYNRKEGEFAINWLVPIGEDSPASIKISVDELDQQRNIIEVPKLYSIDL

SEQ ID NO: 106 - protein, 150 aa, Vibrio cholera
VEEALNIFDECRSPCSLTPEPGKPIQSKLSIPSDVVLDEGVLYYSMTINDEQNDIKDEDKGESIITIGEFATVRATRHYVNQDAPFGVIHLDITTENGTKTYSYNRKEGEFAINWLVPIGEDSPASIKISVDELDQQRNIIEVPKLYSID

SEQ ID NO: 107 - protein, 151 aa, Artificial Sequence
  source: /note="Description of Artificial Sequence: Synthetic polypeptide"
MVEEALNIFDECRSPCSLTPEPGKPIQSKLSIPSDVVLDEGVLYYSMTINDEQNDIKDEDKGESIITIGEFATVRATRHYVNQDAPFGVIHLDITTENGTKTYSYNRKEGEFAINWLVPIGEDSPASIKISVDELDQQRNIIEVPKLYSID

SEQ ID NO: 108 - protein, 149 aa, Vibrio cholera
VEEALNIFDECRSPCSLTPEPGKPIQSKLSIPSDVVLDEGVLYYSMTINDEQNDIKDEDKGESIITIGEFATVRATRHYVNQDAPFGVIHLDITTENGTKTYSYNRKEGEFAINWLVPIGEDSPASIKISVDELDQQRNIIEVPKLYSI

SEQ ID NO: 109 - protein, 148 aa, Vibrio cholera
VEEALNIFDECRSPCSLTPEPGKPIQSKLSIPSDVVLDEGVLYYSMTINDEQNDIKDEDKGESIITIGEFATVRATRHYVNQDAPFGVIHLDITTENGTKTYSYNRKEGEFAINWLVPIGEDSPASIKISVDELDQQRNIIEVPKLYS

SEQ ID NO: 110 - protein, 147 aa, Vibrio cholera
VEEALNIFDECRSPCSLTPEPGKPIQSKLSIPSDVVLDEGVLYYSMTINDEQNDIKDEDKGESIITIGEFATVRATRHYVNQDAPFGVIHLDITTENGTKTYSYNRKEGEFAINWLVPIGEDSPASIKISVDELDQQRNIIEVPKLY

SEQ ID NO: 111 - protein, 146 aa, Vibrio cholera
VEEALNIFDECRSPCSLTPEPGKPIQSKLSIPSDVVLDEGVLYYSMTINDEQNDIKDEDKGESIITIGEFATVRATRHYVNQDAPFGVIHLDITTENGTKTYSYNRKEGEFAINWLVPIGEDSPASIKISVDELDQQRNIIEVPKL

SEQ ID NO: 112 - protein, 145 aa, Vibrio cholera
VEEALNIFDECRSPCSLTPEPGKPIQSKLSIPSDVVLDEGVLYYSMTINDEQNDIKDEDKGESIITIGEFATVRATRHYVNQDAPFGVIHLDITTENGTKTYSYNRKEGEFAINWLVPIGEDSPASIKISVDELDQQRNIIEVPK

SEQ ID NO: 113 - protein, 144 aa, Vibrio cholera
VEEALNIFDECRSPCSLTPEPGKPIQSKLSIPSDVVLDEGVLYYSMTINDEQNDIKDEDKGESIITIGEFATVRATRHYVNQDAPFGVIHLDITTENGTKTYSYNRKEGEFAINWLVPIGEDSPASIKISVDELDQQRNIIEVP

SEQ ID NO: 114 - protein, 143 aa, Vibrio cholera
VEEALNIFDECRSPCSLTPEPGKPIQSKLSIPSDVVLDEGVLYYSMTINDEQNDIKDEDKGESIITIGEFATVRATRHYVNQDAPFGVIHLDITTENGTKTYSYNRKEGEFAINWLVPIGEDSPASIKISVDELDQQRNIIEV

SEQ ID NO: 115 - protein, 142 aa, Vibrio cholera
VEEALNIFDECRSPCSLTPEPGKPIQSKLSIPSDVVLDEGVLYYSMTINDEQNDIKDEDKGESIITIGEFATVRATRHYVNQDAPFGVIHLDITTENGTKTYSYNRKEGEFAINWLVPIGEDSPASIKISVDELDQQRNIIE

SEQ ID NO: 116 - protein, 141 aa, Vibrio cholera
VEEALNIFDECRSPCSLTPEPGKPIQSKLSIPSDVVLDEGVLYYSMTINDEQNDIKDEDKGESIITIGEFATVRATRHYVNQDAPFGVIHLDITTENGTKTYSYNRKEGEFAINWLVPIGEDSPASIKISVDELDQQRNII

SEQ ID NO: 117 - protein, 140 aa, Vibrio cholera
VEEALNIFDECRSPCSLTPEPGKPIQSKLSIPSDVVLDEGVLYYSMTINDEQNDIKDEDKGESIITIGEFATVRATRHYVNQDAPFGVIHLDITTENGTKTYSYNRKEGEFAINWLVPIGEDSPASIKISVDELDQQRNI

SEQ ID NO: 118 - protein, 139 aa, Vibrio cholera
VEEALNIFDECRSPCSLTPEPGKPIQSKLSIPSDVVLDEGVLYYSMTINDEQNDIKDEDKGESIITIGEFATVRATRHYVNQDAPFGVIHLDITTENGTKTYSYNRKEGEFAINWLVPIGEDSPASIKISVDELDQQRN

SEQ ID NO: 119 - protein, 138 aa, Vibrio cholera
VEEALNIFDECRSPCSLTPEPGKPIQSKLSIPSDVVLDEGVLYYSMTINDEQNDIKDEDKGESIITIGEFATVRATRHYVNQDAPFGVIHLDITTENGTKTYSYNRKEGEFAINWLVPIGEDSPASIKISVDELDQQR

SEQ ID NO: 120 - protein, 137 aa, Vibrio cholera
VEEALNIFDECRSPCSLTPEPGKPIQSKLSIPSDVVLDEGVLYYSMTINDEQNDIKDEDKGESIITIGEFATVRATRHYVNQDAPFGVIHLDITTENGTKTYSYNRKEGEFAINWLVPIGEDSPASIKISVDELDQQ

SEQ ID NO: 121 - protein, 136 aa, Vibrio cholera
VEEALNIFDECRSPCSLTPEPGKPIQSKLSIPSDVVLDEGVLYYSMTINDEQNDIKDEDKGESIITIGEFATVRATRHYVNQDAPFGVIHLDITTENGTKTYSYNRKEGEFAINWLVPIGEDSPASIKISVDELDQ

SEQ ID NO: 122 - protein, 135 aa, Vibrio cholera
VEEALNIFDECRSPCSLTPEPGKPIQSKLSIPSDVVLDEGVLYYSMTINDEQNDIKDEDKGESIITIGEFATVRATRHYVNQDAPFGVIHLDITTENGTKTYSYNRKEGEFAINWLVPIGEDSPASIKISVDELD

SEQ ID NO: 123 - protein, 134 aa, Vibrio cholera
VEEALNIFDECRSPCSLTPEPGKPIQSKLSIPSDVVLDEGVLYYSMTINDEQNDIKDEDKGESIITIGEFATVRATRHYVNQDAPFGVIHLDITTENGTKTYSYNRKEGEFAINWLVPIGEDSPASIKISVDEL

SEQ ID NO: 124 - protein, 133 aa, Vibrio cholera
VEEALNIFDECRSPCSLTPEPGKPIQSKLSIPSDVVLDEGVLYYSMTINDEQNDIKDEDKGESIITIGEFATVRATRHYVNQDAPFGVIHLDITTENGTKTYSYNRKEGEFAINWLVPIGEDSPASIKISVDE

SEQ ID NO: 125 - protein, 134 aa, Artificial Sequence
  source: /note="Description of Artificial Sequence: Synthetic polypeptide"
MVEEALNIFDECRSPCSLTPEPGKPIQSKLSIPSDVVLDEGVLYYSMTINDEQNDIKDEDKGESIITIGEFATVRATRHYVNQDAPFGVIHLDITTENGTKTYSYNRKEGEFAINWLVPIGEDSPASIKISVDE

SEQ ID NO: 126 - protein, 121 aa, Vibrio cholera
GNAMSALAAHRVCGVPLETLARSRKPRDLTDDLSCAYQAQNIVSLFVATRILFSHLDSVFTLNLDEQEPEVAERLSDLRRINENNPGMVTQVLTVARQIYNDYVTHHPGLTPEQTSAGAQA

SEQ ID NO: 127 - protein, 39 aa, Vibrio cholera
ADILSLFCPDADKSCVASNNDQANINIESRSGRSYLPEN

SEQ ID NO: 128 - protein, 209 aa, Vibrio cholera
RAVITPQGVTNWTYQELEATHQALTREGYVFVGYHGTNHVAAQTIVNRIAPVPRGNNTENEEKWGGLYVATHAEVAHGYARIKEGTGEYGLPTRAERDARGVMLRVYIPRASLERFYRTNTPLENAEEHITQVIGHSLPLRNEAFTGPESAGGEDETVIGWDMAIHAVAIPSTIPGNAYEELAIDEEAVAKEQSISTKPPYKERKDELK

SEQ ID NO: 129 - protein, 425 aa, Vibrio cholera
VEEALNIFDECRSPCSLTPEPGKPIQSKLSIPSDVVLDEGVLYYSMTINDEQNDIKDEDKGESIITIGEFATVRATRHYVNQDAPFGVIHLDITTENGTKTYSYNRKEGEFAINWLVPIGEDSPASIKISVDELDQQRNIIEVPKLYSIDLDNQTLEQWKTQGNVSFSVTRPEHNIAISWPSVSYKAAQKEGSRHKRWAHWHTGLALCWLVPMDAIYNYITQQNCTLGDNWFGGSYETVAGTPKVITVKQGIEQKPVEQRIHFSKGNAMSALAAHRVCGVPLETLARSRKPRDLTDDLSCAYQAQNIVSLFVATRILFSHLDSVFTLNLDEQEPEVAERLSDLRRINENNPGMVTQVLTVARQIYNDYVTHHPGLTPEQTSAGAQAADILSLFCPDADKSCVASNNDQANINIESRSGRSYLPEN

SEQ ID NO: 130 - protein, 415 aa, Vibrio cholera
VEEALNIFDECRSPCSLTPEPGKPIQSKLSIPSDVVLDEGVLYYSMTINDEQNDIKDEDKGESIITIGEFATVRATRHYVNQDAPFGVIHLDITTENGTKTYSYNRKEGEFAINWLVPIGEDSPASIKISVDELDQQRNIIEVPKLYSIDLDNQTLEQWKTQGNVSFSVTRPEHNIAISWPSVSYKAAQKEGSRHKRWAHWHTGLALCWLVPMDAIYNYITQQNCTLGDNWFGGSYETVAGTPKVITVKQGIEQKPVEQRIHFSKGNAMSALAAHRVCGVPLETLARSRKPRDLTDDLSCAYQAQNIVSLFVATRILFSHLDSVFTLNLDEQEPEVAERLSDLRRINENNPGMVTQVLTVARQIYNDYVTHHPGLTPEQTSAGAQAADILSLFCPDADKSCVASNNDQANINIES

SEQ ID NO: 131 - protein, 397 aa, Vibrio cholera
VEEALNIFDECRSPCSLTPEPGKPIQSKLSIPSDVVLDEGVLYYSMTINDEQNDIKDEDKGESIITIGEFATVRATRHYVNQDAPFGVIHLDITTENGTKTYSYNRKEGEFAINWLVPIGEDSPASIKISVDELDQQRNIIEVPKLYSIDLDNQTLEQWKTQGNVSFSVTRPEHNIAISWPSVSYKAAQKEGSRHKRWAHWHTGLALCWLVPMDAIYNYITQQNCTLGDNWFGGSYETVAGTPKVITVKQGIEQKPVEQRIHFSKGNAMSALAAHRVCGVPLETLARSRKPRDLTDDLSCAYQAQNIVSLFVATRILFSHLDSVFTLNLDEQEPEVAERLSDLRRINENNPGMVTQVLTVARQIYNDYVTHHPGLTPEQTSAGAQAADILSLFCPDA

SEQ ID NO: 132 - protein, 386 aa, Vibrio cholera
VEEALNIFDECRSPCSLTPEPGKPIQSKLSIPSDVVLDEGVLYYSMTINDEQNDIKDEDKGESIITIGEFATVRATRHYVNQDAPFGVIHLDITTENGTKTYSYNRKEGEFAINWLVPIGEDSPASIKISVDELDQQRNIIEVPKLYSIDLDNQTLEQWKTQGNVSFSVTRPEHNIAISWPSVSYKAAQKEGSRHKRWAHWHTGLALCWLVPMDAIYNYITQQNCTLGDNWFGGSYETVAGTPKVITVKQGIEQKPVEQRIHFSKGNAMSALAAHRVCGVPLETLARSRKPRDLTDDLSCAYQAQNIVSLFVATRILFSHLDSVFTLNLDEQEPEVAERLSDLRRINENNPGMVTQVLTVARQIYNDYVTHHPGLTPEQTSAGAQA

SEQ ID NO: 133 - protein, 291 aa, Vibrio cholera
VEEALNIFDECRSPCSLTPEPGKPIQSKLSIPSDVVLDEGVLYYSMTINDEQNDIKDEDKGESIITIGEFATVRATRHYVNQDAPFGVIHLDITTENGTKTYSYNRKEGEFAINWLVPIGEDSPASIKISVDELDQQRNIIEVPKLYSIDLDNQTLEQWKTQGNVSFSVTRPEHNIAISWPSVSYKAAQKEGSRHKRWAHWHTGLALCWLVPMDAIYNYITQQNCTLGDNWFGGSYETVAGTPKVITVKQGIEQKPVEQRIHFSKGNAMSALAAHRVCGVPLETLARSRKP

SEQ ID NO: 134 - DNA, 1902 bp, Vibrio cholera
gtcgaagaagctttaaacatctttgatgaatgccgttcgccatgttcgttgaccccggaaccgggtaagccgattcaatcaaaactgtctatccctagtgatgttgttctggatgaaggtgttctgtattactcgatgacgattaatgatgagcagaatgatattaaggatgaggacaaaggcgagtccattatcactattggtgaatttgccacagtacgcgcgactagacattatgttaatcaagatgcgccttttggtgtcatccatttagatattacgacagaaaatggtacaaaaacgtactcttataaccgcaaagagggtgaatttgcaatcaattggttagtgcctattggtgaagattctcctgcaagcatcaaaatctccgttgatgagctcgatcagcaacgcaatatcatcgaggtgcctaaactgtatagtattgatctcgataaccaaacgttagagcagtggaaaacccaaggtaatgtttctttttcggtaacgcgtcctgaacataatatcgctatctcttggccaagcgtgagttacaaagcagcgcagaaagagggttcacgccataagcgttgggctcattggcatacaggcttagcactgtgttggcttgtgccaatggatgctatctataactatatcacccagcaaaattgtactttaggggataattggtttggtggctcttatgagactgttgcaggcactccgaaggtgattacggttaagcaagggattgaacaaaagccagttgagcagcgcatccatttctccaaggggaatgcgatgagcgcacttgctgctcatcgcgtctgtggtgtgccattagaaactttggcgcgcagtcgcaaacctcgtgatctgacggatgatttatcatgtgcctatcaagcgcagaatatcgtgagtttatttgtcgcgacgcgtatcctgttctctcatctggatagcgtatttactctgaatcttgacgaacaagaaccagaggtggctgaacgtctaagtgatcttcgccgtatcaatgaaaataacccgggcatggttacacaggttttaaccgttgctcgtcagatctataacgattatgtcactcaccatccgggcttaactcctgagcaaaccagtgcgggtgcacaagctgccgatatcctctctttattttgcccagatgctgataagtcttgtgtggcttcaaacaacgatcaagccaatatcaacatcgagtctcgttctggccgttcatatttgcctgaaaaccgtgcggtaatcacccctcaaggcgtcacaaattggacttaccaggaactcgaagcaacacatcaagctctgactcgtgagggttatgtgttcgtgggttaccatggtacgaatcatgtcgctgcgcaaaccatcgtgaatcgcattgcccctgttccgcgcggcaacaacactgaaaacgaggaaaagtggggcgggttatatgttgcaactcacgctgaagttgcccatggttatgctcgcatcaaagaagggacaggggagtatggccttccgacccgtgctgagcgcgacgctcgtggggtaatgctgcgcgtgtatatccctcgtgcttcattagaacgtttttatcgcacgaatacacctttggaaaatgctgaggagcatatcacgcaagtgattggtcattctttgccattacgcaatgaagcatttactggtccagaaagtgcgggcggggaagacgaaactgtcattggctgggatatggcgattcatgcagttgcgatcccttcgactatcccagggaacgcttacgaagaattggcgattgatgaggaggctgttgcaaaagagcaatcgattagcacaaaaccaccttataaagagcgcaaagatgaacttaag

SEQ ID NO: 135 - protein, 613 aa, Pseudomonas aeruginosa
AEEAFDLWNECAKACVLDLKDGVRSSRMSVDPAIADTNGQGVLHYSMVLEGGNDALKLAIDNALSITSDGLTIRLEGGVEPNKPVRYSYTRQARGSWSLNWLVPIGHEKPSNIKVFIHELNAGNQLSHMSPIYTIEMGDELLAKLARDATFFVRAHESNEMQPTLAISHAGVSVVMAQAQPRREKRWSEWASGKVLCLLDPLDGVYNYLAQQRCNLDDTWEGKIYRVLAGNPAKHDLDIKPTVISHRLHFPEGGSLAALTAHQACHLPLETFTRHRQPRGWEQLEQCGYPVQRLVALYLAARLSWNQVDQVIRNALASPGSGGDLGEAIREQPEQARLALTLAAAESERFVRQGTGNDEAGAASADVVSLTCPVAAGECAGPADSGDALLERNYPTGAEFLGDGGDVSFSTRGTQNWTVERLLQAHRQLEERGYVFVGYHGTFLEAAQSIVFGGVRARSQDLDAIWRGFYIAGDPALAYGYAQDQEPDARGRIRNGALLRVYVPRSSLPGFYRTGLTLAAPEAAGEVERLIGHPLPLRLDAITGPEEEGGRLETILGWPLAERTVVIPSAIPTDPRNVGGDLDPSSIPDKEQAISALPDYASQPGKPPREDLK

SEQ ID NO: 136 - DNA, 1839 bp, Pseudomonas aeruginosa
gccgaggaagccttcgacctctggaacgaatgcgccaaggcctgcgtgctcgacctcaaggacggcgtgcgttccagccgcatgagcgtcgacccggccatcgccgacaccaacggccagggcgtgctgcactactccatggtcctggagggcggcaacgacgcgctcaagctggccatcgacaacgccctcagcatcaccagcgacggcctgaccatccgcctcgaaggtggcgtcgagccgaacaagccggtgcgctacagctacacgcgccaggcgcgcggcagttggtcgctgaactggctggtgccgatcggccacgagaagccttcgaacatcaaggtgttcatccacgaactgaacgccggtaaccagctcagccacatgtcgccgatctacaccatcgagatgggcgacgagttgctggcgaagctggcgcgcgatgccaccttcttcgtcagggcgcacgagagcaacgagatgcagccgacgctcgccatcagccatgccggggtcagcgtggtcatggcccaggcccagccgcgccgggaaaagcgctggagcgaatgggccagcggcaaggtgttgtgcctgctcgacccgctggacggggtctacaactacctcgcccagcagcgctgcaacctcgacgatacctgggaaggcaagatctaccgggtgctcgccggcaacccggcgaagcatgacctggacatcaagcccacggtcatcagtcatcgcctgcatttccccgagggcggcagcctggccgcgctgaccgcgcaccaggcctgccacctgccgctggagaccttcacccgtcatcgccagccgcgcggctgggaacaactggagcagtgcggctatccggtgcagcggctggtcgccctctacctggcggcgcggctgtcgtggaaccaggtcgaccaggtgatccgcaacgccctggccagccccggcagcggcggcgacctgggcgaagcgatccgcgagcagccggagcaggcccgtctggccctgaccctggccgccgccgagagcgagcgcttcgtccggcagggcacaggcaacgacgaggccggcgcggccagcgccgacgtggtgagcctgacctgcccggtcgccgccggtgaatgcgcgggcccggcggacagcggcgacgccctgctggagcgcaactatcccactggcgcggagttcctcggcgacggcggcgacatcagcttcagcacccgcggcacgcagaactggacggtggagcggctgctccaggcgcaccgccaactggaggagcgcggctatgtgttcgtcggctaccacggcaccttcctcgaagcggcgcaaagcatcgtcttcggcggggtgcgcgcgcgcagccaggacctcgacgcgatctggcgcggtttctatatcgccggcgatccggcgctggcctacggctacgcccaggaccaggaacccgacgcgcgcggccggatccgcaacggtgccctgctgcgggtctatgtgccgcgctcgagtctgccgggcttctaccgcaccggcctgaccctggccgcgccggaggcggcgggcgaggtcgaacggctgatcggccatccgctgccgctgcgcctggacgccatcaccggccccgaggaggaaggcgggcgcctggaaaccattctcggctggccgctggccgagcgcaccgtggtgattccctcggcgatccccaccgacccgcgcaacgtcggcggcgacctcgacccgtccagcatccccgacaaggaacaggcgatcagcgccctgccggactacgccagccagcccggcaaaccgccgcgcgaggacctgaag

SEQ ID NO: 137 - protein, 252 aa, Pseudomonas aeruginosa
AEEAFDLWNECAKACVLDLKDGVRSSRMSVDPAIADTNGQGVLHYSMVLEGGNDALKLAIDNALSITSDGLTIRLEGGVEPNKPVRYSYTRQARGSWSLNWLVPIGHEKPSNIKVFIHELNAGNQLSHMSPIYTIEMGDELLAKLARDATFFVRAHESNEMQPTLAISHAGVSVVMAQAQPRREKRWSEWASGKVLCLLDPLDGVYNYLAQQRCNLDDTWEGKIYRVLAGNPAKHDLDIKPTVISHRLHFPE

SEQ ID NO: 138 - protein, 112 aa, Pseudomonas aeruginosa
GGSLAALTAHQACHLPLETFTRHRQPRGWEQLEQCGYPVQRLVALYLAARLSWNQVDQVIRNALASPGSGGDLGEAIREQPEQARLALTLAAAESERFVRQGTGNDEAGAAS

SEQ ID NO: 139 - protein, 40 aa, Pseudomonas aeruginosa
ADVVSLTCPVAAGECAGPADSGDALLERNYPTGAEFLGDG

SEQ ID NO: 140 - protein, 209 aa, Pseudomonas aeruginosa
GDVSFSTRGTQNWTVERLLQAHRQLEERGYVFVGYHGTFLEAAQSIVFGGVRARSQDLDAIWRGFYIAGDPALAYGYAQDQEPDARGRIRNGALLRVYVPRSSLPGFYRTGLTLAAPEAAGEVERLIGHPLPLRLDAITGPEEEGGRLETILGWPLAERTVVIPSAIPTDPRNVGGDLDPSSIPDKEQAISALPDYASQPGKPPREDLK

SEQ ID NO: 141 - protein, 404 aa, Pseudomonas aeruginosa
AEEAFDLWNECAKACVLDLKDGVRSSRMSVDPAIADTNGQGVLHYSMVLEGGNDALKLAIDNALSITSDGLTIRLEGGVEPNKPVRYSYTRQARGSWSLNWLVPIGHEKPSNIKVFIHELNAGNQLSHMSPIYTIEMGDELLAKLARDATFFVRAHESNEMQPTLAISHAGVSVVMAQAQPRREKRWSEWASGKVLCLLDPLDGVYNYLAQQRCNLDDTWEGKIYRVLAGNPAKHDLDIKPTVISHRLHFPEGGSLAALTAHQACHLPLETFTRHRQPRGWEQLEQCGYPVQRLVALYLAARLSWNQVDQVIRNALASPGSGGDLGEAIREQPEQARLALTLAAAESERFVRQGTGNDEAGAASADVVSLTCPVAAGECAGPADSGDALLERNYPTGAEFLGDG

SEQ ID NO: 142 - protein, 395 aa, Pseudomonas aeruginosa
AEEAFDLWNECAKACVLDLKDGVRSSRMSVDPAIADTNGQGVLHYSMVLEGGNDALKLAIDNALSITSDGLTIRLEGGVEPNKPVRYSYTRQARGSWSLNWLVPIGHEKPSNIKVFIHELNAGNQLSHMSPIYTIEMGDELLAKLARDATFFVRAHESNEMQPTLAISHAGVSVVMAQAQPRREKRWSEWASGKVLCLLDPLDGVYNYLAQQRCNLDDTWEGKIYRVLAGNPAKHDLDIKPTVISHRLHFPEGGSLAALTAHQACHLPLETFTRHRQPRGWEQLEQCGYPVQRLVALYLAARLSWNQVDQVIRNALASPGSGGDLGEAIREQPEQARLALTLAAAESERFVRQGTGNDEAGAASADVVSLTCPVAAGECAGPADSGDALLERNYP

SEQ ID NO: 143 - protein, 375 aa, Pseudomonas aeruginosa
AEEAFDLWNECAKACVLDLKDGVRSSRMSVDPAIADTNGQGVLHYSMVLEGGNDALKLAIDNALSITSDGLTIRLEGGVEPNKPVRYSYTRQARGSWSLNWLVPIGHEKPSNIKVFIHELNAGNQLSHMSPIYTIEMGDELLAKLARDATFFVRAHESNEMQPTLAISHAGVSVVMAQAQPRREKRWSEWASGKVLCLLDPLDGVYNYLAQQRCNLDDTWEGKIYRVLAGNPAKHDLDIKPTVISHRLHFPEGGSLAALTAHQACHLPLETFTRHRQPRGWEQLEQCGYPVQRLVALYLAARLSWNQVDQVIRNALASPGSGGDLGEAIREQPEQARLALTLAAAESERFVRQGTGNDEAGAASADVVSLTCPVA

SEQ ID NO: 144 - protein, 364 aa, Pseudomonas aeruginosa
AEEAFDLWNECAKACVLDLKDGVRSSRMSVDPAIADTNGQGVLHYSMVLEGGNDALKLAIDNALSITSDGLTIRLEGGVEPNKPVRYSYTRQARGSWSLNWLVPIGHEKPSNIKVFIHELNAGNQLSHMSPIYTIEMGDELLAKLARDATFFVRAHESNEMQPTLAISHAGVSVVMAQAQPRREKRWSEWASGKVLCLLDPLDGVYNYLAQQRCNLDDTWEGKIYRVLAGNPAKHDLDIKPTVISHRLHFPEGGSLAALTAHQACHLPLETFTRHRQPRGWEQLEQCGYPVQRLVALYLAARLSWNQVDQVIRNALASPGSGGDLGEAIREQPEQARLALTLAAAESERFVRQGTGNDEAGAAS

SEQ ID NO: 145 - protein, 277 aa, Pseudomonas aeruginosa
AEEAFDLWNECAKACVLDLKDGVRSSRMSVDPAIADTNGQGVLHYSMVLEGGNDALKLAIDNALSITSDGLTIRLEGGVEPNKPVRYSYTRQARGSWSLNWLVPIGHEKPSNIKVFIHELNAGNQLSHMSPIYTIEMGDELLAKLARDATFFVRAHESNEMQPTLAISHAGVSVVMAQAQPRREKRWSEWASGKVLCLLDPLDGVYNYLAQQRCNLDDTWEGKIYRVLAGNPAKHDLDIKPTVISHRLHFPEGGSLAALTAHQACHLPLETFTRHRQ

SEQ ID NO: 146 - protein, 627 aa, Artificial Sequence
  source: /note="Description of Artificial Sequence: Synthetic polypeptide"
MVEEALNIFDECRSPCSLTPEPGKPIQSKLSIPSDVVLDEGVLYYSMTINDEQNDIKDEDKGESIITIGEFATVRATRHYVNQDAPFGVIHLDITTENGTKTYSYNRKEGEFAINWLVPIGEDSPASIKISVDELDQQRNIIEVPKLYSIDLDNQTLEQWKTQGNVSFSVTRPEHNIAISWPSVSYKAAQKEGSRHKRWAHWHTGLALCWLVPMDAIYNYITQQNCTLGDNWFGGSYETVAGTPKVITVKQGIEQKPVEQRIHFSKGGGSLAALTAHQACHLPLETFTRHRQPRGWEQLEQCGYPVQRLVALYLAARLSWNQVDQVIRNALASPGSGGDLGEAIREQPEQARLALTLAAAESERFVRQGTGNDEAGAASADVVSLTCPVAAGECAGPADSGDALLERNYPTGAEFLGDGGDVSFSTRGTQNWTVERLLQAHRQLEERGYVFVGYHGTFLEAAQSIVFGGVRARSQDLDAIWRGFYIAGDPALAYGYAQDQEPDARGRIRNGALLRVYVPRSSLPGFYRTSLTLAAPEAAGEVERLIGHPLPLRLDAITGPEEEGGRLTILGWPLAERTVVIPSAIPTDPRNVGGDLDPSSIPDKEQAISALPDYASQPGKPPREDLK

SEQ ID NO: 147 - protein, 620 aa, Artificial Sequence
  source: /note="Description of Artificial Sequence: Synthetic polypeptide"
MAEEAFDLWNECAKACVLDLKDGVRSSRMSVDPAIADTNGQGVLHYSMVLEGGNDALKLAIDNALSITSDGLTIRLEGGVEPNKPVRYSYTRQARGSWSLNWLVPIGHEKPSNIKVFIHELNAGNQLSHMSPIYTIEMGDELLAKLARDATFFVRAHESNEMQPTLAISHAGVSVVMAQTQPRREKRWSEWASGKVLCLLDPLDGVYNYLAQQRCNLDDTWEGKIYRVLAGNPAKHDLDIKPTVISHRLHFPEGGNAMSALAAHRVCGVPLETLARSRKPRDLTDDLSCAYQAQNIVSLFVATRILFSHLDSVFTLNLDEQEPEVAERLSDLRRINENNPGMVTQVLTVARQIYNDYVTHHPGLTPEQTSAGAQAAEILSLFCPDADKSCVATNNDQANINIESRSGRSYLPENRAVITPQGVTNWTYQELEATHQALTREGYVFVGYTNHVAAQTIVNRIAPVPRGNNTENEEKWGGLYVATHAEVAHGYARIKEGTGEYGLPTRAERDARGVMLRVYIPRASLERFYRTNTPLENAEEHITQVIGHSLPLRNEAFTGPESAGGEDTVIGWDMAIHAVAIPSTIPGNAYEELAIDEEAVAKEQSISTKPPYKERKDELK

SEQ ID NO: 148 - protein, 18 aa, Vibrio cholera
ELDQQRNIIEVPKLYSID

SEQ ID NO: 149 - protein, 39 aa, Artificial Sequence
  source: /note="Description of Artificial Sequence: Synthetic polypeptide"
MVEEALNIFDECRSPCSLTPEPGKPIQSKLSIPSDVVLD

SEQ ID NO: 150 - protein, 38 aa, Vibrio cholera
VEEALNIFDECRSPCSLTPEPGKPIQSKLSIPSDVVLD

SEQ ID NO: 151 - protein, 37 aa, Vibrio cholera
DLDNQTLEQWKTQGNVSFSVTRPEHNIAISWPSVSYK

SEQ ID NO: 152 - protein, 22 aa, Vibrio cholera
KAAQKEGSRHKRWAHWHTGLAL

SEQ ID NO: 153 - protein, 593 aa, Artificial Sequence
  source: /note="Description of Artificial Sequence: Synthetic polypeptide"
MVEEALNIFDECRSPCSLTPEPGKPIQSKLSIPSDVVLDEGVLYYSMTINDEQNDIKDEDKGESIITIGEFATVRATRHYVNQDAPFGVIHLDITTENGTKTYSYNRKEGEFAINWLVPIGEDSPASIKISVDELDQQRNIIEVPKLYSIDLDNQTLEQWKTQGNVSFSVTRPEHNIAISWPSVSYKAAQKEGSRHKRWAHWHTGLALCWLVPMDAIYNYITQQNCTLGDNWFGGSYETVAGTPKVITVKQGIEQKPVEQRIHFSKGNAMSALAAHRVCGVPLETLARSRKPRDLTDDLSCAYQAQNIVSLFVATRILFSHLDSVFTLNLDEQEPEVAERLSDLRRINENNPGMVTQVLTVARQIYNDYVTHHPGLTPEQTSAGAQAGGGGSGGGGSGGGGSFPTIPLSRLFDNAMLRAHRLHQLAFDTYQEFEEAYIPKEQKYSFLQNPQTSLCFSESIPTPSNREETQQKSNLELLRISLLLIQSWLEPVQFLRSVFANSLVYGASDSNVYDLLKDLEEGIQTLMGRLEDGSPRTGQIFKQTYSKFDTNSHNDDALLKNYGLLYCFRKDMDKVETFLRIVQCRSVEGSCGF

SEQ ID NO: 154 - protein, 580 aa, Artificial Sequence
  source: /note="Description of Artificial Sequence: Synthetic polypeptide"
MVEEALNIFDECRSPCSLTPEPGKPIQSKLSIPSDVVLDEGVLYYSMTINDEQNDIKDEDKGESIITIGEFATVRATRHYVNQDAPFGVIHLDITTENGTKTYSYNRKEGEFAINWLVPIGEDSPASIKISVDELDQQRNIIEVPKLYSIDLDNQTLEQWKTQGNVSFSVTRPEHNIAISWPSVSYKAAQKEGSRHKRWAHWHTGLALCWLVPMDAIYNYITQQNCTLGDNWFGGSYETVAGTPKVITVKQGIEQKPVEQRIHFSKGNAMSALAAHRVCGVPLETLARSRKPRDLTDDLSCAYQAQNIVSLFVATRILFSHLDSVFTLNLDEQEPEVAERLSDLRRINENNPGMVTQVLTVARQIYNDYVTHHPGLTPEQTSAGAQAGGGGSGGGGSGGGGSMHSSALLCCLVLLTGVRASPGQGTQSENSCTHFPGNLPNMLRDLRDAFSRVKTFFQMKDQLDNLLLKESLLEDFKGYLGCQALSEMIQFYLEEVMPQAENQDPDIKAHVNSLGENLKTLRLRLRRCHRFLPCENKSKAVEQVKNAFNKLQEKGIYKAMSEFDIFINYIEAYMTMKIRN

SEQ ID NO: 155 - protein, 460 aa, Artificial Sequence
  source: /note="Description of Artificial Sequence: Synthetic polypeptide"
MVEEALNIFDECRSPCSLTPEPGKPIQSKLSIPSDVVLDEGVLYYSMTINDEQNDIKDEDKGESIITIGEFATVRATRHYVNQDAPFGVIHLDITTENGTKTYSYNRKEGEFAINWLVPIGEDSPASIKISVDELDQQRNIIEVPKLYSIDLDNQTLEQWKTQGNVSFSVTRPEHNIAISWPSVSYKAAQKEGSRHKRWAHWHTGLALCWLVPMDAIYNYITQQNCTLGDNWFGGSYETVAGTPKVITVKQGIEQKPVEQRIHFSKGGGGSGGGGSGGGGSMAALQKSVSSFLMGTLATSCLLLLALLVQGGAAAPISSHCRLDKSNFQQPYITNRTFMLAKEASLADNNTDVRLIGEKLFHGVSMSERCYLMKQVLNFTLEEVLFPQSDRFQPYMQEVVPFLARLSNRLSTCHIEGDDLHIQRNVQKLKDTVKKLGESGEIKAIGELDLLFMSLRNACI

SEQ ID NO: 156 - protein, 491 aa, Artificial Sequence
  source: /note="Description of Artificial Sequence: Synthetic polypeptide"
MVEEALNIFDECRSPCSLTPEPGKPIQSKLSIPSDVVLDEGVLYYSMTINDEQNDIKDEDKGESIITIGEFATVRATRHYVNQDAPFGVIHLDITTENGTKTYSYNRKEGEFAINWLVPIGEDSPASIKISVDELDQQRNIIEVPKLYSIDLDNQTLEQWKTQGNVSFSVTRPEHNIAISWPSVSYKAAQKEGSRHKRWAHWHTGLALCWLVPMDAIYNYITQQNCTLGDNWFGGSYETVAGTPKVITVKQGIEQKPVEQRIHFSKMRSSKNVIKEFMRFKVRMEGTVNGHEFEIEGEGEGRPYEGHNTVKLKVTKGGPLPFAWDILSPQFQYGSKVYVKHPADIPDYKKLSFPEGFKWERVMNFEDGGVVTVTQDSSLQDGCFIYKVKFIGVNFPSDGPVMQKKTMGWEASTERLYPRDGVLKGEIHKALKLKDGGHYLVEFKSIYMAKKPVQLPGYYYVDSKLDITSHNEDYTIVEQYERTEGRHHLFL

SEQ ID NO: 157 - protein, 859 aa, Artificial Sequence
  source: /note="Description of Artificial Sequence: Synthetic polypeptide"
VEDELNIFDECRSPCSLTPEPGKPIQSKLSIPSDVVLDEGVLYYSMTINDEQNDIKDEDKGESIITIGEFATVRATRHYVNQDAPFGVIHLDITTENGTKTYSYNRKEGEFAINWLVPIGEDSPASIKISVDELDQQRNIIEVPKLYSIDLDNQTLEQWKTQGNVSFSVTRPEHNIAISWPSVSYKAAQKEGSRHKRWAHWHTGLALCWLVPMDAIYNYITQQNCTLGDNWFGGSYETVAGTPKVITVKQGIEQKPVEQRIHFSKGNAMSALAAHRVCGVPLETLARSRKPRDLTDDLSCAYQAQNIVSLFVATRILFSHLDSVFTLNLDEQEPEVAERLSDLRRINENNPGMVTQVLTVARQIYNDYVTHHPGLTPEQTSAGAQAADILSLFCPDADKSCVASNNDQANINIESRSGRSYLPENRAVITPQGVTNWTYQELEATHQALTREGYVFVGYHGTNHVAAQTIVNRIAPVPRGNNTENEEKWGGLYVATHAEVAHGYARIKEGTGEYGLPTRAERDARGVMLRVYIPRASLERFYRTNTPLENAEEHITQVIGHSLPLRNEAFTGPESAGGEDATVIGWDMAIHAVAIPSTIPGNAYEELAIDEEAVAKEQSISTKPPYKERKDELKMRSSKNVIKEFMRFKVRMEGTVNGHEFEIEGEGEGRPYEGHNTVKLKVTKGGPLPFAWDILSPQFQYGSKVYVKHPADIPDYKKLSFPEGFKWERVMNFEDGGVVTVTQDSSLQDGCFIYKVKFIGVNFPSDGPVMQKKTMGWEASTERLYPRDGVLKGEIHKALKLKDGGHYLVEFKSIYMAKKPVQLPGYYYVDSKLDITSHNEDYTIVEQYERTEGRHHLFL

SEQ ID NO: 158 - protein, 340 aa, Artificial Sequence
  source: /note="Description of Artificial Sequence: Synthetic polypeptide"
MVEEALNIFDECRSPCSLTPEPGKPIQSKLSIPSDVVLDEGVLYYSMTINDEQNDIKDEDKGESIITIGEFATVRATRHYVNQDAPFGVIHLDITTENGTKTYSYNRKEGEFAINWLVPIGEDSPASIKISVDEGGGGSGGGGSGGGGSFPTIPLSRLFDNAMLRAHRLHQLAFDTYQEFEEAYIPKEQKYSFLQNPQTSLCFSESIPTPSNREETQQKSNLELLRISLLLIQSWLEPVQFLRSVFANSLVYGASDSNVYDLLKDLEEGIQTLMGRLEDGSPRTGQIFKQTYSKFDTNSHNDDALLKNYGLLYCFRKDMDKVETFLRIVQCRSVEGSCGF

SEQ ID NO: 159 - protein, 357 aa, Artificial Sequence
  source: /note="Description of Artificial Sequence: Synthetic polypeptide"
MVEEALNIFDECRSPCSLTPEPGKPIQSKLSIPSDVVLDEGVLYYSMTINDEQNDIKDEDKGESIITIGEFATVRATRHYVNQDAPFGVIHLDITTENGTKTYSYNRKEGEFAINWLVPIGEDSPASIKISVDELDQQRNIIEVPKLYSIDGGGGSGGGGSGGGGSFPTIPLSRLFDNAMLRAHRLHQLAFDTYQEFEEAYIPKEQKYSFLQNPQTSLCFSESIPTPSNREETQQKSNLELLRISLLLIQSWLEPVQFLRSVFANSLVYGASDSNVYDLLKDLEEGIQTLMGRLEDGSPRTGQIFKQTYSKFDTNSHNDDALLKNYGLLYCFRKDMDKVETFLRIVQCRSVEGSCGF

SEQ ID NO: 160 - protein, 393 aa, Artificial Sequence
  source: /note="Description of Artificial Sequence: Synthetic polypeptide"
MVEEALNIFDECRSPCSLTPEPGKPIQSKLSIPSDVVLDEGVLYYSMTINDEQNDIKDEDKGESIITIGEFATVRATRHYVNQDAPFGVIHLDITTENGTKTYSYNRKEGEFAINWLVPIGEDSPASIKISVDELDQQRNIIEVPKLYSIDLDNQTLEQWKTQGNVSFSVTRPEHNIAISWPSVSYKGGGGSGGGGSGGGGSFPTIPLSRLFDNAMLRAHRLHQLAFDTYQEFEEAYIPKEQKYSFLQNPQTSLCFSESIPTPSNREETQQKSNLELLRISLLLIQSWLEPVQFLRSVFANSLVYGASDSNVYDLLKDLEEGIQTLMGRLEDGSPRTGQIFKQTYSKFDTNSHNDDALLKNYGLLYCFRKDMDKVETFLRIVQCRSVEGSCGF

SEQ ID NO: 161 - protein, 412 aa, Artificial Sequence
  source: /note="Description of Artificial Sequence: Synthetic polypeptide"
MVEEALNIFDECRSPCSLTPEPGKPIQSKLSIPSDVVLDEGVLYYSMTINDEQNDIKDEDKGESIITIGEFATVRATRHYVNQDAPFGVIHLDITTENGTKTYSYNRKEGEFAINWLVPIGEDSPASIKISVDELDQQRNIIEVPKLYSIDLDNQTLEQWKTQGNVSFSVTRPEHNIAISWPSVSYKAAQKEGSRHKRWAHWHTGLGGGGSGGGGSGGGGSFPTIPLSRLFDNAMLRAHRLHQLAFDTYQEFEEAYIPKEQKYSFLQNPQTSLCFSESIPTPSNREETQQKSNLELLRISLLLIQSWLEPVQFLRSVFANSLVYGASDSNVYDLLKDLEEGIQTLMGRLEDGSPRTGQIFKQTYSKFDTNSHNDDALLKNYGLLYCFRKDMDKVETFLRIVQCRSVEGSCGF

SEQ ID NO: 162 - protein, 451 aa, Artificial Sequence
  source: /note="Description of Artificial Sequence: Synthetic polypeptide"
MVEEALNIFDECRSPCSLTPEPGKPIQSKLSIPSDVVLDEGVLYYSMTINDEQNDIKDEDKGESIITIGEFATVRATRHYVNQDAPFGVIHLDITTENGTKTYSYNRKEGEFAINWLVPIGEDSPASIKISVDELDQQRNIIEVPKLYSIDLDNQTLEQWKTQGNVSFSVTRPEHNIAISWPSVSYKAAQKEGSRHKRWAHWHTGLALCWLVPMDAIYNYITQQNCTLGDNWFGGSYETVAGTPKGGGGSGGGGSGGGGSFPTIPLSRLFDNAMLRAHRLHQLAFDTYQEFEEAYIPKEQKYSFLQNPQTSLCFSESIPTPSNREETQQKSNLELLRISLLLIQSWLEPVQFLRSVFANSLVYGASDSNVYDLLKDLEEGIQTLMGRLEDGSPRTGQIFKQTYSKFDTNSHNDDALLKNYGLLYCFRKDMDKVETFLRIVQCRSVEGSCGF

SEQ ID NO: 163 - protein, 457 aa, Artificial Sequence
  source: /note="Description of Artificial Sequence: Synthetic polypeptide"
MVEEALNIFDECRSPCSLTPEPGKPIQSKLSIPSDVVLDEGVLYYSMTINDEQNDIKDEDKGESIITIGEFATVRATRHYVNQDAPFGVIHLDITTENGTKTYSYNRKEGEFAINWLVPIGEDSPASIKISVDELDQQRNIIEVPKLYSIDLDNQTLEQWKTQGNVSFSVTRPEHNIAISWPSVSYKAAQKEGSRHKRWAHWHTGLALCWLVPMDAIYNYITQQNCTLGDNWFGGSYETVAGTPKVITVKQGGGGSGGGGSGGGGSFPTIPLSRLFDNAMLRAHRLHQLAFDTYQEFEEAYIPKEQKYSFLQNPQTSLCFSESIPTPSNREETQQKSNLELLRISLLLIQSWLEPVQFLRSVFANSLVYGASDSNVYDLLKDLEEGIQTLMGRLEDGSPRTGQIFKQTYSKFDTNSHNDDALLKNYGLLYCFRKDMDKVETFLRIVQCRSVEGSCGF

SEQ ID NO: 164 - protein, 472 aa, Artificial Sequence
  source: /note="Description of Artificial Sequence: Synthetic polypeptide"
MVEEALNIFDECRSPCSLTPEPGKPIQSKLSIPSDVVLDEGVLYYSMTINDEQNDIKDEDKGESIITIGEFATVRATRHYVNQDAPFGVIHLDITTENGTKTYSYNRKEGEFAINWLVPIGEDSPASIKISVDELDQQRNIIEVPKLYSIDLDNQTLEQWKTQGNVSFSVTRPEHNIAISWPSVSYKAAQKEGSRHKRWAHWHTGLALCWLVPMDAIYNYITQQNCTLGDNWFGGSYETVAGTPKVITVKQGIEQKPVEQRIHFSKGGGGSGGGGSGGGGSFPTIPLSRLFDNAMLRAHRLHQLAFDTYQEFEEAYIPKEQKYSFLQNPQTSLCFSESIPTPSNREETQQKSNLELLRISLLLIQSWLEPVQFLRSVFANSLVYGASDSNVYDLLKDLEEGIQTLMGRLEDGSPRTGQIFKQTYSKFDTNSHNDDALLKNYGLLYCFRKDMDKVETFLRIVQCRSVEGSCGF

SEQ ID NO: 165 - protein, 354 aa, Artificial Sequence
  source: /note="Description of Artificial Sequence: Synthetic polypeptide"
GVLYYSMTINDEQNDIKDEDKGESIITIGEFATVRATRHYVNQDAPFGVIHLDITTENGTKTYSYNRKEGEFAINWLVPIGEDSPASIKISVDELDQQRNIIEVPKLYSIDLDNQTLEQWKTQGNVSFSVTRPEHNIAISWPSVSYKAGGGGSGGGGSGGGGSFPTIPLSRLFDNAMLRAHRLHQLAFDTYQEFEEAYIPKEQKYSFLQNPQTSLCFSESIPTPSNREETQQKSNLELLRISLLLIQSWLEPVQFLRSVFANSLVYGASDSNVYDLLKDLEEGIQTLMGRLEDGSPRTGQIFKQTYSKFDTNSHNDDALLKNYGLLYCFRKDMDKVETFLRIVQCRSVEGSCGF

SEQ ID NO: 166 - protein, 4 aa, Unknown
  source: /note="Description of Unknown: Peptidase cleavage sequence"
AAPF

SEQ ID NO: 167 - protein, 3 aa, Unknown
  source: /note="Description of Unknown: Peptidase cleavage sequence"
GGF

SEQ ID NO: 168 - protein, 4 aa, Unknown
  source: /note="Description of Unknown: Peptidase cleavage sequence"
AAPV

SEQ ID NO: 169 - protein, 3 aa, Unknown
  source: /note="Description of Unknown: Peptidase cleavage sequence"
GGL

SEQ ID NO: 170 - protein, 3 aa, Unknown
  source: /note="Description of Unknown: Peptidase cleavage sequence"
AAL

SEQ ID NO: 171 - protein, 3 aa, Unknown
  source: /note="Description of Unknown: Peptidase cleavage sequence"
FVR

SEQ ID NO: 172 - protein, 3 aa, Unknown
  source: /note="Description of Unknown: Peptidase cleavage sequence"
VGR

SEQ ID NO: 173 - protein, 4 aa, Unknown
  source: /note="Description of Unknown: Peptidase cleavage sequence"
RQPR

SEQ ID NO: 174 - protein, 5 aa, Unknown
  source: /note="Description of Unknown: Peptidase cleavage sequence"
  MOD_RES (5)..(5): Any amino acid
YVADX

SEQ ID NO: 175 - protein, 5 aa, Unknown
  source: /note="Description of Unknown: Peptidase cleavage sequence"
  MOD_RES (2)..(3): Any amino acid
  MOD_RES (5)..(5): Any amino acid
DXXDX

SEQ ID NO: 176 - protein, 9 aa, Unknown
  source: /note="Description of Unknown: Peptidase cleavage sequence"
  MOD_RES (2)..(7): Any amino acid
  SITE (2)..(7): /note="This region may encompass 0, 2, 4 or 6 residues"
  MOD_RES (9)..(9): Any amino acid
RXXXXXXRX

SEQ ID NO: 177 - protein, 9 aa, Unknown
  source: /note="Description of Unknown: Peptidase cleavage sequence"
  MOD_RES (2)..(7): Any amino acid
  SITE (2)..(7): /note="This region may encompass 0, 2, 4 or 6 residues"
  MOD_RES (9)..(9): Any amino acid
KXXXXXXRX

SEQ ID NO: 178 - protein, 6 aa, Unknown
  source: /note="Description of Unknown: Peptidase cleavage sequence"
  MOD_RES (6)..(6): Any amino acid
ERTKRX

SEQ ID NO: 179 - protein, 5 aa, Unknown
  source: /note="Description of Unknown: Peptidase cleavage sequence"
  MOD_RES (5)..(5): Any amino acid
RVRRX

SEQ ID NO: 180 - protein, 5 aa, Unknown
  source: /note="Description of Unknown: Peptidase cleavage sequence"
  MOD_RES (5)..(5): Any amino acid
RVRRX

SEQ ID NO: 181 - protein, 6 aa, Unknown
  source: /note="Description of Unknown: Peptidase cleavage sequence"
  MOD_RES (2)..(2): Any amino acid
  MOD_RES (6)..(6): Any amino acid
PXWVPX

SEQ ID NO: 182 - protein, 4 aa, Unknown
  source: /note="Description of Unknown: Peptidase cleavage sequence"
  MOD_RES (4)..(4): Any amino acid
WVAX

SEQ ID NO: 183 - protein, 4 aa, Unknown
  source: /note="Description of Unknown: Peptidase cleavage sequence"
  MOD_RES (1)..(1): Any amino acid
  MOD_RES (3)..(4): Any amino acid
XFXX

SEQ ID NO: 184 - protein, 4 aa, Unknown
  source: /note="Description of Unknown: Peptidase cleavage sequence"
  MOD_RES (1)..(1): Any amino acid
  MOD_RES (3)..(4): Any amino acid
XYXX

SEQ ID NO: 185 - protein, 4 aa, Unknown
  source: /note="Description of Unknown: Peptidase cleavage sequence"
  MOD_RES (1)..(1): Any amino acid
  MOD_RES (3)..(4): Any amino acid
XWXX

SEQ ID NO: 186 - protein, 12 aa, Unknown
  source: /note="Description of Unknown: Peptidase cleavage sequence"
  VARIANT (10)..(10): /replace="Ala" or "Pro"
  VARIANT (12)..(12): /replace="Pro" or "Ala"
  SITE (1)..(12): /note="Variant residues given in the sequence have no preference with respect to those in the annotations for variant positions"
DRYIPFHLLVYS

SEQ ID NO: 187 - protein, 15 aa, Artificial Sequence
  source: /note="Description of Artificial Sequence: Synthetic peptide"
SGGGGSGKAGSRGLT

SEQ ID NO: 188 - protein, 15 aa, Artificial Sequence
  source: /note="Description of Artificial Sequence: Synthetic peptide"
SGGGGSGGGGLRQPR

SEQ ID NO: 189 - protein, 15 aa, Artificial Sequence
  source: /note="Description of Artificial Sequence: Synthetic peptide"
SGGGGSGKKVERFRY

SEQ ID NO: 190 - protein, 15 aa, Artificial Sequence
  source: /note="Description of Artificial Sequence: Synthetic peptide"
SGGGGSGGGGLMTPR

SEQ ID NO: 191 - protein, 15 aa, Artificial Sequence
  source: /note="Description of Artificial Sequence: Synthetic peptide"
SGGGGSGKAGSFSEG

SEQ ID NO: 192 - protein, 15 aa, Artificial Sequence
  source: /note="Description of Artificial Sequence: Synthetic peptide"
SGGGGSGKAGSAAPF

SEQ ID NO: 193 - protein, 15 aa, Artificial Sequence
  source: /note="Description of Artificial Sequence: Synthetic peptide"
GGGGSGGGENLYFQS

SEQ ID NO: 194 - protein, 12 aa, Artificial Sequence
  source: /note="Description of Artificial Sequence: Synthetic peptide"
VSWKTWFPNLAV

SEQ ID NO: 195 - protein, 12 aa, Artificial Sequence
  source: /note="Description of Artificial Sequence: Synthetic peptide"
YSPFHKWFPSMH

SEQ ID NO: 196 - protein, 12 aa, Artificial Sequence
  source: /note="Description of Artificial Sequence: Synthetic peptide"
IPQVWRDWFKLP

SEQ ID NO: 197 - protein, 12 aa, Artificial Sequence
  source: /note="Description of Artificial Sequence: Synthetic peptide"
FPAWFTKLYPRT

SEQ ID NO: 198 - protein, 12 aa, Artificial Sequence
  source: /note="Description of Artificial Sequence: Synthetic peptide"
QINTAKWWKTHF

SEQ ID NO: 199 - protein, 12 aa, Artificial Sequence
  source: /note="Description of Artificial Sequence: Synthetic peptide"
DASKALRSSGMP

SEQ ID NO: 200 - protein, 6 aa, Artificial Sequence
  source: /note="Description of Artificial Sequence: Synthetic peptide"
WKTWFP

SEQ ID NO: 201 - protein, 15 aa, Artificial Sequence
  source: /note="Description of Artificial Sequence: Synthetic peptide"
SGGGGWKTWFPRGLT

SEQ ID NO: 202 - protein, 15 aa, Artificial Sequence
  source: /note="Description of Artificial Sequence: Synthetic peptide"
SGGGGWKTWFPRQPR

SEQ ID NO: 203 - protein, 15 aa, Artificial Sequence
  source: /note="Description of Artificial Sequence: Synthetic peptide"
SGGGGWKTWFPRFRY

SEQ ID NO: 204 - protein, 15 aa, Artificial Sequence
  source: /note="Description of Artificial Sequence: Synthetic peptide"
SGGGGWKTWFPMTPR

SEQ ID NO: 205 - protein, 15 aa, Artificial Sequence
  source: /note="Description of Artificial Sequence: Synthetic peptide"
SGGGGWKTWFPFSEG

SEQ ID NO: 206 - protein, 15 aa, Artificial Sequence
  source: /note="Description of Artificial Sequence: Synthetic peptide"
SGGGGWKTWFPAAPF

SEQ ID NO: 207 - protein, 5 aa, Artificial Sequence
  source: /note="Description of Artificial Sequence: Synthetic peptide"
GTGGS

SEQ ID NO: 208 - protein, 5 aa, Artificial Sequence
  source: /note="Description of Artificial Sequence: Synthetic peptide"
GGGGS

SEQ ID NO: 209 - protein, 10 aa, Artificial Sequence
  source: /note="Description of Artificial Sequence: Synthetic peptide"
GGGGSGGGGS

SEQ ID NO: 210 - protein, 15 aa, Artificial Sequence
  source: /note="Description of Artificial Sequence: Synthetic peptide"
GGGGSGGGGSGGGGS

SEQ ID NO: 211 - protein, 8 aa, Artificial Sequence
  source: /note="Description of Artificial Sequence: Synthetic peptide"
GGGGSGGG

SEQ ID NO: 212 - protein, 50 aa, Artificial Sequence
  source: /note="Description of Artificial Sequence: Synthetic polypeptide"
  SITE (1)..(50): /note="This sequence may encompass 1-10 'Gly Gly Gly Gly Ser' repeating units"
GGGGSGGGGSGGGGSGGGGSGGGGSGGGGSGGGGSGGGGSGGGGSGGGGS

SEQ ID NO: 213 - protein, 20 aa, Artificial Sequence
  source: /note="Description of Artificial Sequence: Synthetic peptide"
  SITE (1)..(20): /note="This sequence may encompass 1-10 'Gly Ser' repeating units"
GSGSGSGSGSGSGSGSGSGS

SEQ ID NO: 214 - protein, 191 aa, Homo sapiens [sequence omitted]

SEQ ID NO: 215 - protein, 87 aa, Unknown
  source: /note="Description of Unknown: GPL-1 agonist peptide"
MKIILWLCVFGLFLATLFPISWQMPVESGLSSEDSASSESFASKIKRHGEGTFTSDLSKQMEEEAVRLFIEWLKNGGPSSGAPPPSG

SEQ ID NO: 216 - protein, 110 aa, Unknown
  source: /note="Description of Unknown: Insulin peptide"
MALWMRLLPLLALLALWGPDPAAAFVNQHLCGSHLVEALYLVCGERGFFYTPKTRREAEDLQVGQVELGGGPGAGSLQPLALEGSLQKRGIVEQCCTSICSLYQLENYCN

SEQ ID NO: 217 - protein, 178 aa, Homo sapiens
MHSSALLCCLVLLTGVRASPGQGTQSENSCTHFPGNLPNMLRDLRDAFSRVKTFFQMKDQLDNLLLKESLLEDFKGYLGCQALSEMIQFYLEEVMPQAENQDPDIKAHVNSLGENLKTLRLRLRRCHRFLPCENKSKAVEQVKNAFNKLQEKGIYKAMSEFDIFINYIEAYMTMKIRN

SEQ ID NO: 218 - protein, 179 aa, Homo sapiens
MAALQKSVSSFLMGTLATSCLLLLALLVQGGAAAPISSHCRLDKSNFQQPYITNRTFMLAKEASLADNNTDVRLIGEKLFHGVSMSERCYLMKQVLNFTLEEVLFPQSDRFQPYMQEVVPFLARLSNRLSTCHIEGDDLHIQRNVQKLKDTVKKLGESGEIKAIGELDLLFMSLRNACI

SEQ ID NO: 219 - protein, 71 aa, Unknown
  source: /note="Description of Unknown: ExtB polypeptide"
MKKNIAFLLASMFVFSIATNAYASTQSNKKDLCEHYRQIAKESCKKGFLGVRDGTAGACFGAQIMVAAKGC

SEQ ID NO: 220 - protein, 225 aa, Unknown
  source: /note="Description of Unknown: Red Fluorescent Protein (RFP) sequence"
MRSSKNVIKEFMRFKVRMEGTVNGHEFEIEGEGEGRPYEGHNTVKLKVTKGGPLPFAWDILSPQFQYGSKVYVKHPADIPDYKKLSFPEGFKWERVMNFEDGGVVTVTQDSSLQDGCFIYKVKFIGVNFPSDGPVMQKKTMGWEASTERLYPRDGVLKGEIHKALKLKDGGHYLVEFKSIYMAKKPVQLPGYYYVDSKLDITSHNEDYTIVEQYERTEGRHHLFL

SEQ ID NO: 221 - protein, 281 aa, Artificial Sequence
  source: /note="Description of Artificial Sequence: Synthetic polypeptide"
MVEEALNIFDECRSPCSLTPEPGKPIQSKLSIPSDVVLDEGVLYYSMTINDEQNDIKDEDKGESIITIGEFATVRATRHYVNQDAPFGVIHLDITTENGTKTYSYNRKEGEFAINWLVPIGEDSPASIKISVDELDQQRNIIEVPKLYSIDLDNQTLEQWKTQGNVSFSVTRPEHNIAISWPSVSYKAAQKEGSRHKRWAHWHTGLALCWLVPMDAIYNYITQQNCTLGDNWFGGSYETVAGTPKVITVKQGIEQKPVEQRIHFSKGGGGSGGGGSGGGGS